European Patent Application EP 4 223 317 A2, published August 9, 2023. Title: MODULATION OF COMPLEMENT ACTIVITY. Applicant: RA Pharmaceuticals, Inc. The sequence listing filed with the application follows.

SEQUENCE LISTING (212 sequences)

SEQ ID NO: 1 - protein, 13 aa, synthetic construct
  REGION 1..13: note = Description of Artificial Sequence: Synthetic peptide
  REGION 1..13: note = N-term Ac
  MOD_RES 1: note = Nvl
  MOD_RES 8: note = 7-azatryptophan
  MOD_RES 12: note = Tbg
  REGION 1..13: note = C-term NH2
VCYKNYHWEYPGY

SEQ ID NO: 2 - protein, 13 aa, synthetic construct
  REGION 1..13: note = Description of Artificial Sequence: Synthetic peptide
  REGION 1..13: note = N-term Ac
  MOD_RES 1: note = Nvl
  MOD_RES 6: note = Tbg
  MOD_RES 8: note = 7-azatryptophan
  MOD_RES 11: note = (N-Me)Gly
  MOD_RES 12: note = Nvl
  MOD_RES 13: note = (N-Me)Ser
  REGION 1..13: note = C-term NH2
VCYENGYWEYGVS

SEQ ID NO: 3 - protein, 13 aa, synthetic construct
  REGION 1..13: note = Description of Artificial Sequence: Synthetic peptide
  REGION 1..13: note = N-term Ac
  MOD_RES 1: note = Nvl
  MOD_RES 6: note = Tbg
  MOD_RES 8: note = 7-azatryptophan
  MOD_RES 12: note = Phg
  MOD_RES 13: note = Nvl
  REGION 1..13: note = C-term NH2
VCYENGYWEYPGV

SEQ ID NO: 4 - protein, 13 aa, synthetic construct
  REGION 1..13: note = Description of Artificial Sequence: Synthetic peptide
  REGION 1..13: note = N-term Ac
  MOD_RES 1: note = Nvl
  MOD_RES 6: note = Tbg
  MOD_RES 8: note = 7-azatryptophan
  MOD_RES 12: note = Phg
  REGION 1..13: note = C-term NH2
VCYENGYWEYPGP

SEQ ID NO: 5 - protein, 13 aa, synthetic construct
  REGION 1..13: note = Description of Artificial Sequence: Synthetic peptide
  REGION 1..13: note = N-term Ac
  MOD_RES 1: note = Nvl
  MOD_RES 6: note = Tbg
  MOD_RES 8: note = 7-azatryptophan
  MOD_RES 12: note = Phg
  MOD_RES 13: note = Tbg
  REGION 1..13: note = C-term NH2
VCYNNGEWEYPGG

SEQ ID NO: 6 - protein, 13 aa, synthetic construct
  REGION 1..13: note = Description of Artificial Sequence: Synthetic peptide
  REGION 1..13: note = N-term Ac
  MOD_RES 1: note = Nvl
  MOD_RES 4: note = 7-azatryptophan
  MOD_RES 5: note = (N-Me)Gly
  MOD_RES 6: note = Tbg
  MOD_RES 7: note = Nvl
  MOD_RES 8: note = 7-azatryptophan
  MOD_RES 12: note = Phg
  REGION 1..13: note = C-term NH2
VCYWGGVWEYPGP

SEQ ID NO: 7 - protein, 11 aa, synthetic construct
  REGION 1..11: note = Description of Artificial Sequence: Synthetic peptide
  REGION 1..11: note = N-term Ac
  MOD_RES 4: note = Tbg
  MOD_RES 6: note = 7-azatryptophan
  MOD_RES 9: note = (N-Me)Gly
  MOD_RES 10: note = Nvl
  MOD_RES 11: note = (N-Me)Ser
  REGION 1..11: note = C-term NH2
YENGYWEYGVS

SEQ ID NO: 8 - protein, 13 aa, synthetic construct
  REGION 1..13: note = Description of Artificial Sequence: Synthetic peptide
  REGION 1..13: note = N-term Ac
  MOD_RES 1: note = Nvl
  REGION 2..7: note = misc_feature - Bridging moiety between residues
  MOD_RES 5: note = Phg
  MOD_RES 8: note = (N-Me)Ser
  MOD_RES 9: note = Tbg
  MOD_RES 11: note = 7-azatryptophan
  REGION 1..13: note = C-term NH2
VCKEGYCSGKWEY

SEQ ID NO: 9 - protein, 13 aa, synthetic construct
  REGION 1..13: note = Description of Artificial Sequence: Synthetic peptide
  REGION 1..13: note = N-term Ac
  MOD_RES 1: note = Nvl
  REGION 2..10: note = misc_feature - Bridging moiety between residues
  MOD_RES 3: note = Phg
  MOD_RES 5: note = 7-azatryptophan
  MOD_RES 8: note = (N-Me)Ser
  MOD_RES 11: note = Nvl
  MOD_RES 13: note = Nvl
  REGION 1..13: note = C-term NH2
VCGTWEYSHCVPV

SEQ ID NO: 10 - protein, 13 aa, synthetic construct
  REGION 1..13: note = Description of Artificial Sequence: Synthetic peptide
  REGION 2..7: note = misc_feature - Bridging moiety between residues
  REGION 1..13: note = C-term NH2
MCSERYCEVRWEY

SEQ ID NO: 11 - protein, 13 aa, synthetic construct
  REGION 1..13: note = Description of Artificial Sequence: Synthetic peptide
  REGION 2..7: note = misc_feature - Bridging moiety between residues
  REGION 1..13: note = C-term NH2
MCVERFCDVYWEF

SEQ ID NO: 12 - protein, 13 aa, synthetic construct
  REGION 1..13: note = Description of Artificial Sequence: Synthetic peptide
  MOD_RES 1..2: note = Nvl
  MOD_RES 6: note = Tbg
  MOD_RES 8: note = 7-azatryptophan
  MOD_RES 12: note = Phg
  MOD_RES 13: note = Nvl
  REGION 1..13: note = C-term NH2
VVYENGYWEYPGV

SEQ ID NO: 13 - protein, 13 aa, synthetic construct
  REGION 1..13: note = Description of Artificial Sequence: Synthetic peptide
  REGION 1..13: note = N-term Ac
  MOD_RES 1: note = Nvl
  MOD_RES 6: note = Tbg
  MOD_RES 8: note = 7-azatryptophan
  MOD_RES 12: note = Phg
  MOD_RES 13: note = Nvl
  REGION 1..13: note = C-term NH2
VSYENGYWEYPGV

SEQ ID NO: 14 - protein, 13 aa, synthetic construct
  REGION 1..13: note = Description of Artificial Sequence: Synthetic peptide
  REGION 1..13: note = N-term Ac
  MOD_RES 1..2: note = Nvl
  MOD_RES 5: note = (N-Me)Asn
  MOD_RES 6: note = Tbg
  MOD_RES 8: note = 7-azatryptophan
  MOD_RES 12: note = Chg
  MOD_RES 13: note = Nvl
  REGION 1..13: note = C-term NH2
VVYENGYWEYPGV

SEQ ID NO: 15 - protein, 16 aa, synthetic construct
  REGION 1..16: note = Description of Artificial Sequence: Synthetic peptide
  REGION 2..7: note = misc_feature - Bridging moiety between residues
  MOD_RES 9: note = Tbg
  MOD_RES 11: note = 7-azatryptophan
  MOD_RES 15: note = Phg
  MOD_RES 16: note = Nvl
  REGION 1..16: note = C-term NH2
MCVERFCDGYWEYPGV

SEQ ID NO: 16 - protein, 13 aa, synthetic construct
  REGION 1..13: note = Description of Artificial Sequence: Synthetic peptide
  REGION 1..13: note = N-term Ac
  MOD_RES 1..2: note = Nvl
  MOD_RES 6: note = Tbg
  MOD_RES 8: note = 7-azatryptophan
  MOD_RES 12: note = Phg
  MOD_RES 13: note = Nvl
  REGION 1..13: note = C-term NH2
VVYENGYWEYPGV

SEQ ID NO: 17 - protein, 13 aa, synthetic construct
  REGION 1..13: note = Description of Artificial Sequence: Synthetic peptide
  REGION 1..13: note = N-term Ac
  MOD_RES 1: note = Nvl
  MOD_RES 6: note = Tbg
  MOD_RES 8: note = 7-azatryptophan
  MOD_RES 12: note = Chg
  MOD_RES 13: note = Nvl
  REGION 1..13: note = C-term NH2
VCYENGYWEYPGV

SEQ ID NO: 18 - protein, 12 aa, synthetic construct
  REGION 1..12: note = Description of Artificial Sequence: Synthetic peptide
  REGION 1..12: note = N-term Ac
  MOD_RES 1: note = Nvl
  MOD_RES 6: note = Tbg
  MOD_RES 8: note = 7-azatryptophan
  MOD_RES 12: note = Phg
  REGION 1..12: note = C-term NH2
VCYENGYWEYPG

SEQ ID NO: 19 - protein, 12 aa, synthetic construct
  REGION 1..12: note = Description of Artificial Sequence: Synthetic peptide
  REGION 1..12: note = N-term Ac
  REGION 1..6: note = misc_feature - Bridging moiety between residues
  REGION 1..12: note = C-term NH2
CVERFCDVYWEF

SEQ ID NO: 20 - protein, 14 aa, synthetic construct
  REGION 1..14: note = Description of Artificial Sequence: Synthetic peptide
  REGION 1..14: note = N-term Ac
  MOD_RES 1..2: note = Nvl
  MOD_RES 6: note = Tbg
  MOD_RES 8: note = 7-azatryptophan
  MOD_RES 12: note = Chg
  MOD_RES 13: note = Nvl
  REGION 1..14: note = C-term NH2
VVYENGYWEYPGVK

SEQ ID NO: 21 - protein, 12 aa, synthetic construct
  REGION 1..12: note = Description of Artificial Sequence: Synthetic peptide
  REGION 1..12: note = N-term Ac
  MOD_RES 5: note = Tbg
  MOD_RES 7: note = 7-azatryptophan
  MOD_RES 11: note = Phg
  MOD_RES 12: note = Nvl
  REGION 1..12: note = C-term NH2
CYENGYWEYPGV

SEQ ID NO: 22 - protein, 13 aa, synthetic construct
  REGION 1..13: note = Description of Artificial Sequence: Synthetic peptide
  REGION 1..13: note = N-term Ac
  MOD_RES 1..2: note = Nvl
  MOD_RES 3: note = (N-Me)Tyr
  MOD_RES 6: note = Tbg
  MOD_RES 8: note = 7-azatryptophan
  MOD_RES 12: note = Chg
  MOD_RES 13: note = Nvl
  REGION 1..13: note = C-term NH2
VVYENGYWEYPGV

SEQ ID NO: 23 - protein, 11 aa, synthetic construct
  REGION 1..11: note = Description of Artificial Sequence: Synthetic peptide
  REGION 1..11: note = N-term Ac
  MOD_RES 1: note = Nvl
  REGION 2..10: note = misc_feature - Bridging moiety between residues
  MOD_RES 3: note = Phg
  MOD_RES 5: note = 7-azatryptophan
  MOD_RES 8: note = (N-Me)Ser
  MOD_RES 11: note = Nvl
  REGION 1..11: note = C-term NH2
VCGTWEYSHCV

SEQ ID NO: 24 - protein, 11 aa, synthetic construct
  REGION 1..11: note = Description of Artificial Sequence: Synthetic peptide
  REGION 1..11: note = N-term Ac
  MOD_RES 4: note = Tbg
  MOD_RES 6: note = 7-azatryptophan
  MOD_RES 10: note = Phg
  MOD_RES 11: note = Nvl
  REGION 1..11: note = C-term NH2
YENGYWEYPGV

SEQ ID NO: 25 - protein, 13 aa, synthetic construct
  REGION 1..13: note = Description of Artificial Sequence: Synthetic peptide
  REGION 1..13: note = N-term Ac
  MOD_RES 1: note = Nvl
  MOD_RES 6: note = Tbg
  MOD_RES 8: note = 7-azatryptophan
  MOD_RES 12: note = Chg
  MOD_RES 13: note = Nvl
  REGION 1..13: note = C-term NH2
VSYEAGYWEYPGV

SEQ ID NO: 26 - protein, 11 aa, synthetic construct
  REGION 1..11: note = Description of Artificial Sequence: Synthetic peptide
  REGION 1..11: note = N-term Ac
  MOD_RES 4: note = Tbg
  MOD_RES 10: note = Phg
  MOD_RES 11: note = Nvl
  REGION 1..11: note = C-term NH2
YENGYWEYPGV

SEQ ID NO: 27 - protein, 14 aa, synthetic construct
  REGION 1..14: note = Description of Artificial Sequence: Synthetic peptide
  REGION 1..14: note = N-term Ac
  MOD_RES 1..2: note = Nvl
  MOD_RES 6: note = Tbg
  MOD_RES 8: note = 7-azatryptophan
  MOD_RES 12: note = Chg
  MOD_RES 13: note = Nvl
  REGION 1..14: note = C-term (PEG2000)NH2
VVYENGYWEYPGVK

SEQ ID NO: 28 - protein, 11 aa, synthetic construct
  REGION 1..11: note = Description of Artificial Sequence: Synthetic peptide
  REGION 1..11: note = N-term Ac
  MOD_RES 1: note = Nvl
  MOD_RES 6: note = Tbg
  MOD_RES 8: note = 7-azatryptophan
  REGION 1..11: note = C-term NH2
VCYENGYWEYP

SEQ ID NO: 29 - protein, 13 aa, synthetic construct
  REGION 1..13: note = Description of Artificial Sequence: Synthetic peptide
  REGION 1..13: note = N-term Ac
  MOD_RES 1: note = Nvl
  MOD_RES 8: note = 7-azatryptophan
  MOD_RES 12: note = Chg
  MOD_RES 13: note = Nvl
  REGION 1..13: note = C-term NH2
VSYENAYWEYPGV

SEQ ID NO: 30 - protein, 13 aa, synthetic construct
  REGION 1..13: note = Description of Artificial Sequence: Synthetic peptide
  REGION 1..13: note = N-term Ac
  MOD_RES 1: note = Nvl
  MOD_RES 6: note = Tbg
  MOD_RES 8: note = 7-azatryptophan
  MOD_RES 12: note = Chg
  MOD_RES 13: note = Nvl
  REGION 1..13: note = C-term NH2
VSYENGAWEYPGV

SEQ ID NO: 31 - protein, 12 aa, synthetic construct
  REGION 1..12: note = Description of Artificial Sequence: Synthetic peptide
  REGION 1..12: note = N-term Ac
  MOD_RES 1: note = Nvl
  REGION 2..10: note = misc_feature - Bridging moiety between residues
  MOD_RES 3: note = Phg
  MOD_RES 5: note = 7-azatryptophan
  MOD_RES 8: note = (N-Me)Ser
  MOD_RES 11: note = Nvl
  REGION 1..12: note = C-term NH2
VCGTWEYSHCVP

SEQ ID NO: 32 - protein, 13 aa, synthetic construct
  REGION 1..13: note = Description of Artificial Sequence: Synthetic peptide
  REGION 1..13: note = N-term Ac
  MOD_RES 1: note = Nvl
  MOD_RES 6: note = Tbg
  MOD_RES 8: note = 7-azatryptophan
  MOD_RES 12: note = Chg
  MOD_RES 13: note = Nvl
  REGION 1..13: note = C-term NH2
VSYENGYWEYAGV

SEQ ID NO: 33 - protein, 13 aa, synthetic construct
  REGION 1..13: note = Description of Artificial Sequence: Synthetic peptide
  REGION 1..13: note = N-term Ac
  MOD_RES 1: note = Nvl
  MOD_RES 6: note = Tbg
  MOD_RES 8: note = 7-azatryptophan
  MOD_RES 13: note = Nvl
  REGION 1..13: note = C-term NH2
VSYENGYWEYPAV

SEQ ID NO: 34 - protein, 11 aa, synthetic construct
  REGION 1..11: note = Description of Artificial Sequence: Synthetic peptide
  REGION 1..11: note = N-term Ac
  MOD_RES 1: note = Nvl
  REGION 2..10: note = misc_feature - Bridging moiety between residues
  MOD_RES 3: note = Phg
  MOD_RES 5: note = 7-azatryptophan
  MOD_RES 8: note = (N-Me)Ser
  MOD_RES 11: note = Nvl
  REGION 1..11: note = C-term NH2
VCGAWEYSHCV

SEQ ID NO: 35 - protein, 11 aa, synthetic construct
  REGION 1..11: note = Description of Artificial Sequence: Synthetic peptide
  REGION 1..11: note = N-term Ac
  MOD_RES 1: note = Nvl
  REGION 2..10: note = misc_feature - Bridging moiety between residues
  MOD_RES 3: note = Phg
  MOD_RES 5: note = 7-azatryptophan
  MOD_RES 8: note = (N-Me)Ser
  MOD_RES 11: note = Nvl
  REGION 1..11: note = C-term NH2
VCGTWEYSACV

SEQ ID NO: 36 - protein, 11 aa, synthetic construct
  REGION 1..11: note = Description of Artificial Sequence: Synthetic peptide
  REGION 1..11: note = N-term Ac
  MOD_RES 1: note = Nvl
  REGION 2..10: note = misc_feature - Bridging moiety between residues
  MOD_RES 3: note = Phg
  MOD_RES 5: note = 7-azatryptophan
  MOD_RES 8: note = (N-Me)Ser
  MOD_RES 11: note = Nvl
  REGION 1..11: note = C-term NH2
VCGTWEYSHCV

SEQ ID NO: 37 - protein, 13 aa, synthetic construct
  REGION 1..13: note = Description of Artificial Sequence: Synthetic peptide
  REGION 1..13: note = N-term Ac
  MOD_RES 1: note = Nvl
  MOD_RES 6: note = Tbg
  MOD_RES 8: note = 7-azatryptophan
  MOD_RES 12: note = Chg
  MOD_RES 13: note = Nvl
  REGION 1..13: note = C-term NH2
VSYANGYWEYPGV

SEQ ID NO: 38 - protein, 11 aa, synthetic construct
  REGION 1..11: note = Description of Artificial Sequence: Synthetic peptide
  REGION 1..11: note = N-term Ac
  MOD_RES 1: note = Nvl
  REGION 2..10: note = misc_feature - Bridging moiety between residues
  MOD_RES 3: note = Phg
  MOD_RES 5: note = 7-azatryptophan
  MOD_RES 8: note = (N-Me)Ser
  REGION 1..11: note = C-term NH2
VCGTWEYSHCA

SEQ ID NO: 39 - protein, 11 aa, synthetic construct
  REGION 1..11: note = Description of Artificial Sequence: Synthetic peptide
  REGION 1..11: note = N-term Ac
  MOD_RES 1: note = Nvl
  REGION 2..10: note = misc_feature - Bridging moiety between residues
  MOD_RES 3: note = Phg
  MOD_RES 5: note = 7-azatryptophan
  MOD_RES 8: note = (N-Me)Ala
  MOD_RES 11: note = Nvl
  REGION 1..11: note = C-term NH2
VCGTWEYAHCV

SEQ ID NO: 40 - protein, 14 aa, synthetic construct
  REGION 1..14: note = Description of Artificial Sequence: Synthetic peptide
  REGION 1..14: note = N-term Ac
  MOD_RES 1..2: note = Nvl
  MOD_RES 6: note = Tbg
  MOD_RES 8: note = 7-azatryptophan
  MOD_RES 12: note = Chg
  MOD_RES 13: note = Nvl
  REGION 1..14: note = C-term (BODIPY-TMR-X)NH2
VVYENGYWEYPGVK

SEQ ID NO: 41 - protein, 11 aa, synthetic construct
  REGION 1..11: note = Description of Artificial Sequence: Synthetic peptide
  REGION 1..11: note = N-term Ac
  MOD_RES 1: note = Nvl
  REGION 2..10: note = misc_feature - Bridging moiety between residues
  MOD_RES 3: note = Phg
  MOD_RES 5: note = 7-azatryptophan
  MOD_RES 7: note = Tyr(OMe)
  MOD_RES 8: note = (N-Me)Ser
  MOD_RES 11: note = Nvl
  REGION 1..11: note = C-term NH2
VCGTWEYSHCV

SEQ ID NO: 42 - protein, 10 aa, synthetic construct
  REGION 1..10: note = Description of Artificial Sequence: Synthetic peptide
  REGION 1..10: note = N-term Ac
  MOD_RES 1: note = Nvl
  REGION 2..10: note = misc_feature - Bridging moiety between residues
  MOD_RES 3: note = Phg
  MOD_RES 5: note = 7-azatryptophan
  MOD_RES 8: note = (N-Me)Ser
  REGION 1..10: note = C-term NH2
VCGTWEYSHC

SEQ ID NO: 43 - protein, 11 aa, synthetic construct
  REGION 1..11: note = Description of Artificial Sequence: Synthetic peptide
  REGION 1..11: note = N-term Ac
  MOD_RES 1: note = Nvl
  REGION 2..10: note = misc_feature - Bridging moiety between residues
  MOD_RES 3: note = Phg
  MOD_RES 5: note = 7-azatryptophan
  MOD_RES 11: note = Nvl
  REGION 1..11: note = C-term NH2
VCGTWEYPHCV

SEQ ID NO: 44 - protein, 11 aa, synthetic construct
  REGION 1..11: note = Description of Artificial Sequence: Synthetic peptide
  REGION 1..11: note = N-term Ac
  MOD_RES 1: note = Nvl
  REGION 2..10: note = misc_feature - Bridging moiety between residues
  MOD_RES 3: note = Phg
  MOD_RES 5: note = 7-azatryptophan
  MOD_RES 7: note = Phe(4-F)
  MOD_RES 8: note = (N-Me)Ser
  MOD_RES 11: note = Nvl
  REGION 1..11: note = C-term NH2
VCGTWEFSHCV

SEQ ID NO: 45 - protein, 13 aa, synthetic construct
  REGION 1..13: note = Description of Artificial Sequence: Synthetic peptide
  REGION 1..13: note = N-term Ac
  MOD_RES 1..2: note = Nvl
  MOD_RES 6: note = Tbg
  MOD_RES 8: note = (N-Me)Trp
  MOD_RES 12: note = Chg
  MOD_RES 13: note = Nvl
  REGION 1..13: note = C-term NH2
VVYENGYWEYPGV

SEQ ID NO: 46 - protein, 11 aa, synthetic construct
  REGION 1..11: note = Description of Artificial Sequence: Synthetic peptide
  REGION 1..11: note = N-term Ac
  MOD_RES 1: note = Nvl
  REGION 2..10: note = misc_feature - Bridging moiety between residues
  MOD_RES 3: note = Phg
  MOD_RES 8: note = (N-Me)Ser
  MOD_RES 11: note = Nvl
  REGION 1..11: note = C-term NH2
VCGTWEYSACV

SEQ ID NO: 47 - protein, 13 aa, synthetic construct
  REGION 1..13: note = Description of Artificial Sequence: Synthetic peptide
  REGION 1..13: note = N-term PEG2000
  MOD_RES 1..2: note = Nvl
  MOD_RES 6: note = Tbg
  MOD_RES 8: note = 7-azatryptophan
  MOD_RES 12: note = Phg
  MOD_RES 13: note = Nvl
  REGION 1..13: note = C-term NH2
VVYENGYWEYPGV

SEQ ID NO: 48 - protein, 11 aa, synthetic construct
  REGION 1..11: note = Description of Artificial Sequence: Synthetic peptide
  REGION 1..11: note = N-term Ac
  MOD_RES 1: note = Nvl
  REGION 2..10: note = misc_feature - Bridging moiety between residues
  MOD_RES 3: note = Phg
  MOD_RES 5: note = 7-azatryptophan
  MOD_RES 8: note = (N-Me)Ser
  MOD_RES 11: note = Nvl
  REGION 1..11: note = C-term NH2
VCGTWEFSACV

SEQ ID NO: 49 - protein, 13 aa, synthetic construct
  REGION 1..13: note = Description of Artificial Sequence: Synthetic peptide
  REGION 1..13: note = N-term Ac
  MOD_RES 1..2: note = Nvl
  MOD_RES 6: note = Tbg
  MOD_RES 8: note = 7-azatryptophan
  MOD_RES 12: note = (N-Me)Phg
  MOD_RES 13: note = Nvl
  REGION 1..13: note = C-term NH2
VVYENGYWEYPGV

SEQ ID NO: 50 - protein, 12 aa, synthetic construct
  REGION 1..12: note = Description of Artificial Sequence: Synthetic peptide
  REGION 2..7: note = misc_feature - Bridging moiety between residues
  REGION 1..12: note = C-term NH2
MCVERFCDVYWE

SEQ ID NO: 51 - protein, 11 aa, synthetic construct
  REGION 1..11: note = Description of Artificial Sequence: Synthetic peptide
  REGION 1..11: note = N-term Ac
  MOD_RES 1: note = Nvl
  REGION 2..10: note = misc_feature - Bridging moiety between residues
  MOD_RES 3: note = Phg
  MOD_RES 5: note = 7-azatryptophan
  MOD_RES 11: note = Nvl
  REGION 1..11: note = C-term NH2
VCGTWEYPHCV

SEQ ID NO: 52 - protein, 10 aa, synthetic construct
  REGION 1..10: note = Description of Artificial Sequence: Synthetic peptide
  REGION 1..10: note = N-term Ac
  MOD_RES 3: note = Tbg
  MOD_RES 5: note = 7-azatryptophan
  MOD_RES 9: note = Phg
  MOD_RES 10: note = Nvl
  REGION 1..10: note = C-term NH2
ENGYWEYPGV

SEQ ID NO: 53 - protein, 11 aa, synthetic construct
  REGION 1..11: note = Description of Artificial Sequence: Synthetic peptide
  REGION 1..11: note = N-term Ac
  REGION 2..10: note = misc_feature - Bridging moiety between residues
  MOD_RES 3: note = Phg
  MOD_RES 5: note = 7-azatryptophan
  MOD_RES 8: note = (N-Me)Ser
  MOD_RES 11: note = Nvl
  REGION 1..11: note = C-term NH2
ACGTWEYSHCV

SEQ ID NO: 54 - protein, 14 aa, synthetic construct
  REGION 1..14: note = Description of Artificial Sequence: Synthetic peptide
  REGION 1..14: note = N-term Ac
  MOD_RES 1: note = Nvl
  REGION 2..14: note = misc_feature - Bridging moiety between residues
  MOD_RES 6: note = Tbg
  MOD_RES 8: note = 7-azatryptophan
  MOD_RES 12: note = Phg
  MOD_RES 13: note = Nvl
  REGION 1..14: note = C-term NH2
VCYENGYWEYPGVC

SEQ ID NO: 55 - protein, 12 aa, synthetic construct
  REGION 1..12: note = Description of Artificial Sequence: Synthetic peptide
  REGION 1..12: note = N-term Ac
  REGION 1..9: note = misc_feature - Bridging moiety between residues
  MOD_RES 2: note = Phg
  MOD_RES 4: note = 7-azatryptophan
  MOD_RES 7: note = (N-Me)Ser
  MOD_RES 10: note = Nvl
  MOD_RES 12: note = Nvl
  REGION 1..12: note = C-term NH2
CGTWEYSHCVPV

SEQ ID NO: 56 - protein, 11 aa, synthetic construct
  REGION 1..11: note = Description of Artificial Sequence: Synthetic peptide
  REGION 1..11: note = N-term Ac
  MOD_RES 1: note = Nvl
  REGION 2..10: note = misc_feature - Bridging moiety between residues
  MOD_RES 2: note = HomoCys
  MOD_RES 3: note = Phg
  MOD_RES 5: note = 7-azatryptophan
  MOD_RES 8: note = (N-Me)Ser
  MOD_RES 11: note = Nvl
  REGION 1..11: note = C-term NH2
VCGTWEYSHCV

SEQ ID NO: 57 - protein, 13 aa, synthetic construct
  REGION 1..13: note = Description of Artificial Sequence: Synthetic peptide
  REGION 1..13: note = N-term Ac
  MOD_RES 1: note = Nvl
  MOD_RES 6: note = Tbg
  MOD_RES 8: note = 7-azatryptophan
  MOD_RES 12: note = Chg
  MOD_RES 13: note = Nvl
  REGION 1..13: note = C-term NH2
VSAENGYWEYPGV

SEQ ID NO: 58 - protein, 13 aa, synthetic construct
  REGION 1..13: note = Description of Artificial Sequence: Synthetic peptide
  REGION 1..13: note = N-term Ac
  MOD_RES 1..2: note = Nvl
  MOD_RES 4: note = (N-Me)Glu
  MOD_RES 6: note = Tbg
  MOD_RES 8: note = 7-azatryptophan
  MOD_RES 12: note = Chg
  MOD_RES 13: note = Nvl
  REGION 1..13: note = C-term NH2
VVYENGYWEYPGV

SEQ ID NO: 59 - protein, 11 aa, synthetic construct
  REGION 1..11: note = Description of Artificial Sequence: Synthetic peptide
  REGION 1..11: note = N-term Ac
  MOD_RES 4: note = Tbg
  MOD_RES 6: note = (1-Me)Trp
  MOD_RES 10: note = Phg
  MOD_RES 11: note = Nvl
  REGION 1..11: note = C-term NH2
YENGYWEYPGV

SEQ ID NO: 60 - protein, 13 aa, synthetic construct
  REGION 1..13: note = Description of Artificial Sequence: Synthetic peptide
  REGION 1..13: note = N-term Ac
  MOD_RES 1: note = Nvl
  MOD_RES 6: note = Tbg
  MOD_RES 8: note = 7-azatryptophan
  MOD_RES 12: note = Phg
  MOD_RES 13: note = Tbg
  REGION 1..13: note = C-term NH2
VCYNNGEWECPGG

SEQ ID NO: 61 - protein, 11 aa, synthetic construct
  REGION 1..11: note = Description of Artificial Sequence: Synthetic peptide
  REGION 1..11: note = N-term Ac
  MOD_RES 1: note = Nvl
  REGION 2..10: note = misc_feature - Bridging moiety between residues
  MOD_RES 3: note = Phg
  MOD_RES 5: note = 7-azatryptophan
  MOD_RES 8: note = (N-Me)Ser
  MOD_RES 11: note = Nvl
  REGION 1..11: note = C-term NH2
VCGTWEYSHCV

SEQ ID NO: 62 - protein, 13 aa, synthetic construct
  REGION 1..13: note = Description of Artificial Sequence: Synthetic peptide
  REGION 1..13: note = N-term Ac
  MOD_RES 1: note = Nvl
  MOD_RES 6: note = Tbg
  MOD_RES 8: note = 7-azatryptophan
  MOD_RES 12: note = Chg
  MOD_RES 13: note = Nvl
  REGION 1..13: note = C-term NH2
VSYENGYWEAPGV

SEQ ID NO: 63 - protein, 9 aa, synthetic construct
  REGION 1..9: note = Description of Artificial Sequence: Synthetic peptide
  REGION 1..9: note = N-term Ac
  REGION 1..9: note = misc_feature - Bridging moiety between residues
  MOD_RES 2: note = Phg
  MOD_RES 4: note = 7-azatryptophan
  MOD_RES 7: note = (N-Me)Ser
  REGION 1..9: note = C-term NH2
CGTWEYSHC

SEQ ID NO: 64 - protein, 13 aa, synthetic construct
  REGION 1..13: note = Description of Artificial Sequence: Synthetic peptide
  REGION 1..13: note = N-term Ac
  MOD_RES 1: note = Nvl
  MOD_RES 6: note = Tbg
  MOD_RES 8: note = 7-azatryptophan
  MOD_RES 12: note = Chg
  MOD_RES 13: note = Nvl
  REGION 1..13: note = C-term NH2
VSYENGYWAYPGV

SEQ ID NO: 65 - protein, 11 aa, synthetic construct
  REGION 1..11: note = Description of Artificial Sequence: Synthetic peptide
  REGION 1..11: note = N-term Ac
  MOD_RES 1: note = Nvl
  REGION 2..10: note = misc_feature - Bridging moiety between residues
  MOD_RES 3: note = Phg
  MOD_RES 5: note = 7-azatryptophan
  MOD_RES 8: note = (N-Me)Ser
  MOD_RES 10: note = HomoCys
  MOD_RES 11: note = Nvl
  REGION 1..11: note = C-term NH2
VCGTWEYSHCV

SEQ ID NO: 66 - protein, 11 aa, synthetic construct
  REGION 1..11: note = Description of Artificial Sequence: Synthetic peptide
  REGION 1..11: note = N-term Ac
  MOD_RES 1: note = Nvl
  REGION 2..10: note = misc_feature - Bridging moiety between residues
  MOD_RES 3: note = Phg
  MOD_RES 5: note = 7-azatryptophan
  MOD_RES 8: note = (N-Me)Ser
  MOD_RES 10: note = HomoCys
  MOD_RES 11: note = Nvl
  REGION 1..11: note = C-term NH2
VCGTWEYSHCV

SEQ ID NO: 67 - protein, 11 aa, synthetic construct
  REGION 1..11: note = Description of Artificial Sequence: Synthetic peptide
  REGION 1..11: note = N-term Ac
  MOD_RES 1: note = Nvl
  MOD_RES 3: note = Phg
  REGION 4..10: note = misc_feature - Bridging moiety between residues
  MOD_RES 5: note = 7-azatryptophan
  MOD_RES 8: note = (N-Me)Ser
  MOD_RES 11: note = Nvl
  REGION 1..11: note = C-term NH2
VTGCWEYSACV

SEQ ID NO: 68 - protein, 11 aa, synthetic construct
  REGION 1..11: note = Description of Artificial Sequence: Synthetic peptide
  REGION 1..11: note = N-term Ac
  MOD_RES 1: note = Nle
  REGION 2..10: note = misc_feature - Bridging moiety between residues
  MOD_RES 3: note = Phg
  MOD_RES 5: note = 7-azatryptophan
  MOD_RES 8: note = (N-Me)Ser
  MOD_RES 11: note = Nvl
  REGION 1..11: note = C-term NH2
LCGTWEYSHCV

SEQ ID NO: 69 - protein, 12 aa, synthetic construct
  REGION 1..12: note = Description of Artificial Sequence: Synthetic peptide
  REGION 1..12: note = N-term Ac
  MOD_RES 2: note = Nvl
  REGION 3..11: note = misc_feature - Bridging moiety between residues
  MOD_RES 4: note = Phg
  MOD_RES 6: note = 7-azatryptophan
  MOD_RES 9: note = (N-Me)Ser
  MOD_RES 12: note = Nvl
  REGION 1..12: note = C-term NH2
YVCGTWEYSHCV

SEQ ID NO: 70 - protein, 11 aa, synthetic construct
  REGION 1..11: note = Description of Artificial Sequence: Synthetic peptide
  REGION 1..11: note = N-term Ac
  MOD_RES 1: note = Nvl
  REGION 2..10: note = misc_feature - Bridging moiety between residues
  MOD_RES 3: note = Phg
  MOD_RES 5: note = 7-azatryptophan
  MOD_RES 7: note = (3-Cl-Phe)
  MOD_RES 8: note = (N-Me)Ser
  MOD_RES 11: note = Nvl
  REGION 1..11: note = C-term NH2
VCGTWEFSACV

SEQ ID NO: 71 - protein, 13 aa, synthetic construct
  REGION 1..13: note = Description of Artificial Sequence: Synthetic peptide
  REGION 1..13: note = N-term Ac
  MOD_RES 1: note = Nvl
  REGION 2..10: note = misc_feature - Bridging moiety between residues
  MOD_RES 6: note = Tbg
  MOD_RES 8: note = 7-azatryptophan
  MOD_RES 12: note = Phg
  MOD_RES 13: note = Nvl
  REGION 1..13: note = C-term NH2
VCYENGYWECPGV

SEQ ID NO: 72 - protein, 9 aa, synthetic construct
  REGION 1..9: note = Description of Artificial Sequence: Synthetic peptide
  REGION 1..9: note = N-term Ac
  MOD_RES 2: note = Tbg
  MOD_RES 4: note = 7-azatryptophan
  MOD_RES 8: note = Phg
  MOD_RES 9: note = Nvl
  REGION 1..9: note = C-term NH2
NGYWEYPGV

SEQ ID NO: 73 - protein, 8 aa, synthetic construct
  REGION 1..8: note = Description of Artificial Sequence: Synthetic peptide
  REGION 1..8: note = N-term Ac
  MOD_RES 1: note = Tbg
  MOD_RES 3: note = 7-azatryptophan
  MOD_RES 7: note = Phg
  MOD_RES 8: note = Nvl
  REGION 1..8: note = C-term NH2
GYWEYPGV

SEQ ID NO: 74 - protein, 11 aa, synthetic construct
  REGION 1..11: note = Description of Artificial Sequence: Synthetic peptide
  REGION 1..11: note = N-term Ac
  MOD_RES 1: note = Nvl
  REGION 2..10: note = misc_feature - Bridging moiety between residues
  MOD_RES 5: note = 7-azatryptophan
  MOD_RES 8: note = (N-Me)Ser
  MOD_RES 11: note = Nvl
  REGION 1..11: note = C-term NH2
VCATWEYSHCV

SEQ ID NO: 75 - protein, 11 aa, synthetic construct
  REGION 1..11: note = Description of Artificial Sequence: Synthetic peptide
  REGION 1..11: note = N-term Ac
  MOD_RES 1: note = Nvl
  REGION 2..10: note = misc_feature - Bridging moiety between residues
  MOD_RES 3: note = Chg
  MOD_RES 5: note = 7-azatryptophan
  MOD_RES 8: note = (N-Me)Ser
  MOD_RES 11: note = Nvl
  REGION 1..11: note = C-term NH2
VCGTWEYSHCV

SEQ ID NO: 76 - protein, 13 aa, synthetic construct
  REGION 1..13: note = Description of Artificial Sequence: Synthetic peptide
  REGION 1..13: note = N-term Ac
  MOD_RES 1: note = Nvl
  MOD_RES 6: note = Tbg
  MOD_RES 12: note = Chg
  MOD_RES 13: note = Nvl
  REGION 1..13: note = C-term NH2
VSYENGYAEYPGV

SEQ ID NO: 77 - protein, 13 aa, synthetic construct
  REGION 1..13: note = Description of Artificial Sequence: Synthetic peptide
  REGION 1..13: note = N-term Ac
  MOD_RES 1..2: note = Nvl
  MOD_RES 6: note = Tbg
  MOD_RES 8: note = 7-azatryptophan
  MOD_RES 10: note = (N-Me)Tyr
  MOD_RES 12: note = Chg
  MOD_RES 13: note = Nvl
  REGION 1..13: note = C-term NH2
VVYENGYWEYPGV

SEQ ID NO: 78 - protein, 13 aa, synthetic construct
  REGION 1..13: note = Description of Artificial Sequence: Synthetic peptide
  REGION 1..13: note = N-term Ac
  MOD_RES 1: note = Nvl
  MOD_RES 3: note = Phg
  MOD_RES 5: note = 7-azatryptophan
  MOD_RES 8: note = (N-Me)Ser
  MOD_RES 11: note = Nvl
  MOD_RES 13: note = Nvl
  REGION 1..13: note = C-term NH2
VCGTWEYSHCVPV

SEQ ID NO: 79 - protein, 9 aa, synthetic construct
  REGION 1..9: note = Description of Artificial Sequence: Synthetic peptide
  REGION 1..9: note = N-term Ac
  REGION 1..9: note = misc_feature - Bridging moiety between residues
  MOD_RES 2: note = Tbg
  MOD_RES 4: note = 7-azatryptophan
  MOD_RES 7: note = (N-Me)Ser
  REGION 1..9: note = C-term NH2
CGYWEYSHC

SEQ ID NO: 80 - protein, 11 aa, synthetic construct
  REGION 1..11: note = Description of Artificial Sequence: Synthetic peptide
  REGION 1..11: note = N-term Ac
  MOD_RES 1: note = Chg
  REGION 2..10: note = misc_feature - Bridging moiety between residues
  MOD_RES 3: note = Phg
  MOD_RES 5: note = 7-azatryptophan
  MOD_RES 8: note = (N-Me)Ser
  MOD_RES 11: note = Nvl
  REGION 1..11: note = C-term NH2
GCGTWEYSACV

SEQ ID NO: 81 - protein, 11 aa, synthetic construct
  REGION 1..11: note = Description of Artificial Sequence: Synthetic peptide
  REGION 1..11: note = N-term Ac
  REGION 2..10: note = misc_feature - Bridging moiety between residues
  MOD_RES 3: note = Phg
  MOD_RES 5: note = 7-azatryptophan
  MOD_RES 8: note = (N-Me)Ser
  MOD_RES 11: note = Nvl
  REGION 1..11: note = C-term NH2
VCGTWEYSACV

SEQ ID NO: 82 - protein, 11 aa, synthetic construct
  REGION 1..11: note = Description of Artificial Sequence: Synthetic peptide
  REGION 1..11: note = N-term Ac
  MOD_RES 1: note = Nvl
  REGION 2..10: note = misc_feature - Bridging moiety between residues
  MOD_RES 3: note = (2-OMe)Phg
  MOD_RES 5: note = 7-azatryptophan
  MOD_RES 8: note = (N-Me)Ser
  MOD_RES 11: note = Nvl
  REGION 1..11: note = C-term NH2
VCGTWEYSHCV

SEQ ID NO: 83 - protein, 11 aa, synthetic construct
  REGION 1..11: note = Description of Artificial Sequence: Synthetic peptide
  REGION 1..11: note = N-term Ac
  MOD_RES 1: note = Nvl
  MOD_RES 2: note = HomoCys
  REGION 2..10: note = misc_feature - Bridging moiety between residues
  MOD_RES 3: note = Phg
  MOD_RES 5: note = 7-azatryptophan
  MOD_RES 8: note = (N-Me)Ser
  MOD_RES 11: note = Nvl
  REGION 1..11: note = C-term NH2
VCGTWEYSHCV

SEQ ID NO: 84 - protein, 11 aa, synthetic construct
  REGION 1..11: note = Description of Artificial Sequence: Synthetic peptide
  REGION 1..11: note = N-term Ac
  MOD_RES 1: note = Nvl
  REGION 2..10: note = misc_feature - Bridging moiety between residues
  MOD_RES 3: note = Phg
  MOD_RES 5: note = 7-azatryptophan
  MOD_RES 8: note = (N-Me)Ser
  MOD_RES 9: note = D-Ala
  MOD_RES 11: note = Nvl
  REGION 1..11: note = C-term NH2
VCGTWEYSACV

SEQ ID NO: 85 - protein, 11 aa, synthetic construct
  REGION 1..11: note = Description of Artificial Sequence: Synthetic peptide
  REGION 1..11: note = N-term Ac
  MOD_RES 1: note = Nvl
  REGION 2..10: note = misc_feature - Bridging moiety between residues
  MOD_RES 3: note = Phg
  MOD_RES 8: note = (N-Me)Ser
  MOD_RES 11: note = Nvl
  REGION 1..11: note = C-term NH2
VCGTAEYSHCV

SEQ ID NO: 86 - protein, 11 aa, synthetic construct
  REGION 1..11: note = Description of Artificial Sequence: Synthetic peptide
  REGION 1..11: note = N-term Ac
  MOD_RES 1: note = Nvl
  REGION 2..10: note = misc_feature - Bridging moiety between residues
  MOD_RES 3: note = Phg
  MOD_RES 5: note = 7-azatryptophan
  MOD_RES 8: note = (N-Me)Ser
  MOD_RES 11: note = Nvl
  REGION 1..11: note = C-term NH2
VCGTWAYSHCV

SEQ ID NO: 87 - protein, 11 aa, synthetic construct
  REGION 1..11: note = Description of Artificial Sequence: Synthetic peptide
  REGION 1..11: note = N-term Ac
  MOD_RES 1: note = Nvl
  REGION 2..10: note = misc_feature - Bridging moiety between residues
  MOD_RES 3: note = Phg
  MOD_RES 5: note = 7-azatryptophan
  MOD_RES 8: note = (N-Me)Ser
  MOD_RES 11: note = Nvl
  REGION 1..11: note = C-term NH2
VCGTWEASHCV

SEQ ID NO: 88 - protein, 11 aa, synthetic construct
  REGION 1..11: note = Description of Artificial Sequence: Synthetic peptide
  REGION 2..7: note = misc_feature - Bridging moiety between residues
  REGION 1..11: note = C-term NH2
MCVERFCDVYW

SEQ ID NO: 89 - protein, 10 aa, synthetic construct
  REGION 1..10: note = Description of Artificial Sequence: Synthetic peptide
  REGION 1..10: note = N-term Ac
  MOD_RES 1: note = Nvl
  REGION 2..9: note = misc_feature - Bridging moiety between residues
  MOD_RES 3: note = Phg
  MOD_RES 5: note = 7-azatryptophan
  MOD_RES 8: note = (N-Me)Ser
  MOD_RES 10: note = Nvl
  REGION 1..10: note = C-term NH2
VCGTWEYSCV

SEQ ID NO: 90 - protein, 11 aa, synthetic construct
  REGION 1..11: note = Description of Artificial Sequence: Synthetic peptide
  REGION 1..11: note = N-term heptanoyl
  MOD_RES 1: note = Nvl
  REGION 2..10: note = misc_feature - Bridging moiety between residues
  MOD_RES 3: note = Phg
  MOD_RES 5: note = 7-azatryptophan
  MOD_RES 8: note = (N-Me)Ser
  MOD_RES 11: note = Nvl
  REGION 1..11: note = C-term NH2
VCGTWEYSACV

SEQ ID NO: 91 - protein, 14 aa, synthetic construct
  REGION 1..14: note = Description of Artificial Sequence: Synthetic peptide
  REGION 1..14: note = N-term Ac
  MOD_RES 1: note = Nvl
  REGION 5..13: note = misc_feature - Bridging moiety between residues
  MOD_RES 6: note = Tbg
  MOD_RES 8: note = 7-azatryptophan
  MOD_RES 12: note = Chg
  MOD_RES 14: note = Nvl
  REGION 1..14: note = C-term NH2
VSYECGYWEYPGCV

SEQ ID NO: 92 - protein, 11 aa, synthetic construct
  REGION 1..11: note = Description of Artificial Sequence: Synthetic peptide
  REGION 1..11: note = N-term Ac
  MOD_RES 1: note = Nvl
  REGION 2..10: note = misc_feature - Bridging moiety between residues
  MOD_RES 3: note = Phg
  MOD_RES 8: note = (N-Me)Ser
  MOD_RES 11: note = Nvl
  REGION 1..11: note = C-term NH2
VCGTFEYSACV

SEQ ID NO: 93 - protein, 11 aa, synthetic construct
  REGION 1..11: note = Description of Artificial Sequence: Synthetic peptide
  REGION 1..11: note = N-term Ac
  MOD_RES 1: note = Nvl
  REGION 2..10: note = misc_feature - Bridging moiety between residues
  MOD_RES 3: note = Phg
  MOD_RES 5: note = 7-azatryptophan
  MOD_RES 7: note = (Homo)Phe
  MOD_RES 8: note = (N-Me)Ser
  MOD_RES 11: note = Nvl
  REGION 1..11: note = C-term NH2
VCGTWEFSACV

SEQ ID NO: 94 - protein, 11 aa, synthetic construct
  REGION 1..11: note = Description of Artificial Sequence: Synthetic peptide
  REGION 1..11: note = N-term Ac
  MOD_RES 1: note = Nvl
  REGION 2..10: note = misc_feature - Bridging moiety between residues
  MOD_RES 3: note = Phg
  MOD_RES 4: note = Aib
  MOD_RES 5: note = 7-azatryptophan
  MOD_RES 8: note = (N-Me)Ser
  MOD_RES 11: note = Nvl
  REGION 1..11: note = C-term NH2
VCGXWEYSHCV

SEQ ID NO: 95 - protein, 11 aa, synthetic construct
  REGION 1..11: note = Description of Artificial Sequence: Synthetic peptide
  REGION 1..11: note = N-term Ac
  MOD_RES 1: note = Nvl
  REGION 2..10: note = misc_feature - Bridging moiety between residues
  MOD_RES 3: note = Tiq
  MOD_RES 5: note = 7-azatryptophan
  MOD_RES 8: note = (N-Me)Ser
  MOD_RES 11: note = Nvl
  REGION 1..11: note = C-term NH2
VCXTWEYSHCV

SEQ ID NO: 96 - protein, 11 aa, synthetic construct
  REGION 1..11: note = Description of Artificial Sequence: Synthetic peptide
  MOD_RES 1: note = Nvl
  REGION 2..11: note = misc_feature - Bridging moiety between residues
  MOD_RES 4: note = (N-Me)Ser
  MOD_RES 5: note = Phg
  MOD_RES 6: note = 4-F-(N-Me)Phe
  MOD_RES 7: note = (N-Me)Ser
  MOD_RES 9: note = 4-F-(N-Me)Phe
  REGION 1..11: note = C-term NH2
VCYSGFSHFGC

SEQ ID NO: 97 - protein, 11 aa, synthetic construct
  REGION 1..11: note = Description of Artificial Sequence: Synthetic peptide
  REGION 1..11: note = N-term Ac
  MOD_RES 1: note = Nvl
  MOD_RES 2: note = HomoCys
  REGION 2..10: note = misc_feature - Bridging moiety between residues
  MOD_RES 3: note = Phg
  MOD_RES 5: note = 7-azatryptophan
  MOD_RES 8: note = (N-Me)Ser
  MOD_RES 10: note = HomoCys
  MOD_RES 11: note = Nvl
  REGION 1..11: note = C-term NH2
VCGTWEYSHCV

SEQ ID NO: 98 - protein, 11 aa, synthetic construct
  REGION 1..11: note = Description of Artificial Sequence: Synthetic peptide
  REGION 1..11: note = N-term Ac
  MOD_RES 1: note = Nvl
  MOD_RES 2: note = HomoCys
  REGION 2..10: note = misc_feature - Bridging moiety between residues
  MOD_RES 3: note = Phg
  MOD_RES 5: note = 7-azatryptophan
  MOD_RES 8: note = (N-Me)Ser
  MOD_RES 10: note = HomoCys
  MOD_RES 11: note = Nvl
  REGION 1..11: note = C-term NH2
VCGTWEYSHCV

SEQ ID NO: 99 - protein, 13 aa, synthetic construct
  REGION 1..13: note = Description of Artificial Sequence: Synthetic peptide
  REGION 1..13: note = N-term Ac
  MOD_RES 1: note = Nvl
  REGION 2..10: note = misc_feature - Bridging moiety between residues
  MOD_RES 6: note = Tbg
  MOD_RES 8: note = 7-azatryptophan
  MOD_RES 12: note = Phg
  MOD_RES 13: note = Tbg
  REGION 1..13: note = C-term NH2
VCYNNGEWECPGG

SEQ ID NO: 100 - protein, 11 aa, synthetic construct
  REGION 1..11: note = Description of Artificial Sequence: Synthetic peptide
  REGION 1..11: note = N-term Ac
  MOD_RES 1: note = Nvl
  REGION 2..10: note = misc_feature - Bridging moiety between residues
  MOD_RES 3: note = Phg
  MOD_RES 4: note = D-Ala
  MOD_RES 5: note = 7-azatryptophan
  MOD_RES 8: note = (N-Me)Ser
  MOD_RES 11: note = Nvl
  REGION 1..11: note = C-term NH2
VCGAWEYSHCV

SEQ ID NO: 101 - protein, 13 aa, synthetic construct
  REGION 1..13: note = Description of Artificial Sequence: Synthetic peptide
  REGION 1..13: note = N-term Ac
  MOD_RES 1: note = Nvl
  REGION 2..10: note = misc_feature - Bridging moiety between residues
  MOD_RES 5: note = (N-Me)Gly
  MOD_RES 6: note = Tbg
  MOD_RES 8: note = 7-azatryptophan
  MOD_RES 11: note = Nvl
  MOD_RES 13: note = Nvl
  REGION 1..13: note = C-term NH2
VCYEGGYWECVPV

SEQ ID NO: 102 - protein, 13 aa, synthetic construct
  REGION 1..13: note = Description of Artificial Sequence: Synthetic peptide
  REGION 1..13: note = N-term Ac
  MOD_RES 1: note = Nvl
  REGION 2..13: note = misc_feature - Bridging moiety between residues
  MOD_RES 5: note = (N-Me)Gly
  MOD_RES 6: note = Tbg
  MOD_RES 8: note = 7-azatryptophan
  MOD_RES 10..11: note = Nvl
  REGION 1..13: note = C-term NH2
VCYEGGYWEVVPC

SEQ ID NO: 103 - protein, 13 aa, synthetic construct
  REGION 1..13: note = Description of Artificial Sequence: Synthetic peptide
  REGION 1..13: note = N-term Ac
  MOD_RES 1: note = Nvl
  REGION 2..8: note = misc_feature - Bridging moiety between residues
  MOD_RES 6: note = Tbg
  MOD_RES 12: note = Phg
  MOD_RES 13: note = Nvl
  REGION 1..13: note = C-term NH2
VCYENGYCEYPGV

SEQ ID NO: 104 - protein, 13 aa, synthetic construct
  REGION 1..13: note = Description of Artificial Sequence: Synthetic peptide
  REGION 1..13: note = N-term Ac
  MOD_RES 5: note = Phg
  MOD_RES 6: note = 7-azatryptophan
  MOD_RES 7: note = Tbg
  MOD_RES 9: note = Nvl
  MOD_RES 12: note = Nvl
  REGION 1..13: note = C-term NH2
YPYCGWGEVNYVE

SEQ ID NO: 105 - protein, 13 aa, synthetic construct
  REGION 1..13: note = Description of Artificial Sequence: Synthetic peptide
  REGION 1..13: note = N-term Ac
  MOD_RES 1: note = Nvl
  REGION 2..10: note = misc_feature - Bridging moiety between residues
  MOD_RES 3: note = Phg
  MOD_RES 5: note = 7-azatryptophan
  MOD_RES 8: note = (N-Me)Ser
  MOD_RES 11: note = Nvl
  MOD_RES 13: note = Nvl
VCGTWEYSHCVPV

SEQ ID NO: 106 - protein, 11 aa, synthetic construct
  REGION 1..11: note = Description of Artificial Sequence: Synthetic peptide
  REGION 1..11: note = N-term Ac
  MOD_RES 1: note = Nvl
  REGION 2..10: note = misc_feature - Bridging moiety between residues
  MOD_RES 3: note = Phg
  MOD_RES 5: note = 7-azatryptophan
  MOD_RES 8: note = (N-Me)Ser
  MOD_RES 11: note = Nvl
  REGION 1..11: note = C-term NH2
VCGTWEYSHCV

SEQ ID NO: 107 - protein, 10 aa, synthetic construct
  REGION 1..10: note = Description of Artificial Sequence: Synthetic peptide
  REGION 2..7: note = misc_feature - Bridging moiety between residues
  REGION 1..10: note = C-term NH2
MCVERFCDVY

SEQ ID NO: 108 - protein, 9 aa, synthetic construct
  REGION 1..9: note = Description of Artificial Sequence: Synthetic peptide
  REGION 2..7: note = misc_feature - Bridging moiety between residues
  REGION 1..9: note = C-term NH2
MCVERFCDV

SEQ ID NO: 109 - protein, 7 aa, synthetic construct
  REGION 1..7: note = Description of Artificial Sequence: Synthetic peptide
  REGION 2..7: note = misc_feature - Bridging moiety between residues
  REGION 1..7: note = C-term NH2
MCVERFC

SEQ ID NO: 110 - protein, 11 aa, synthetic construct
  REGION 1..11: note = Description of Artificial Sequence: Synthetic peptide
  MOD_RES 1: note = Nvl
  REGION 2..11: note = misc_feature - Bridging moiety between residues
  MOD_RES 4: note = (N-Me)Ser
  MOD_RES 5: note = Phg
  MOD_RES 6: note = 4-F-(N-Me)Phe
  MOD_RES 7: note = (N-Me)Ser
  MOD_RES 9: note = 4-F-(N-Me)Phe
  MOD_RES 10: note = (N-Me)Gly
  REGION 1..11: note = C-term NH2
VCYSGFSHFGC

SEQ ID NO: 111 - protein, 11 aa, synthetic construct
  REGION 1..11: note = Description of Artificial Sequence: Synthetic peptide
  MOD_RES 1: note = Nvl
  REGION 2..9: note = misc_feature - Bridging moiety between residues
  MOD_RES 4: note = Tbg
  MOD_RES 5: note = Phg
  MOD_RES 7: note = (N-Me)Gly
  MOD_RES 10: note = Phg
  MOD_RES 11: note = (N-Me)Ala
  REGION 1..11: note = C-term NH2
VCYGGNGLCGA

SEQ ID NO: 112 - protein, 11 aa, synthetic construct
  REGION 1..11: note = Description of Artificial Sequence: Synthetic peptide
  REGION 1..11: note = misc_feature - Bicyclic peptide
  MOD_RES 1: note = Nvl
  MOD_RES 5: note = Tbg
  MOD_RES 6: note = Phg
  MOD_RES 8: note = Tbg
  MOD_RES 9: note = (N-Me)Ser
  MOD_RES 11: note = Tbg
  REGION 1..11: note = C-term NH2
VCCNGGCGSCG

SEQ ID NO: 113 - protein, 5 aa, synthetic construct
  REGION 1..5: note = Description of Artificial Sequence: Synthetic peptide
  REGION 1..5: note = N-term Ac
  MOD_RES 1: note = Tbg
  MOD_RES 3: note = 7-azatryptophan
  REGION 1..5: note = C-term NH2
GYWEY

SEQ ID NO: 114 - protein, 5 aa, synthetic construct
  REGION 1..5: note = Description of Artificial Sequence: Synthetic peptide
  REGION 1..5: note = N-term Ac
  MOD_RES 2: note = 7-azatryptophan
  REGION 1..5: note = C-term NH2
YWEYP

SEQ ID NO: 115 - protein, 11 aa, synthetic construct
  REGION 1..11: note = Description of Artificial Sequence: Synthetic peptide
  REGION 1..11: note = N-term Ac
  MOD_RES 4: note = Tbg
  MOD_RES 6: note = 7-azatryptophan
  MOD_RES 7: note = (N-Me)Glu
  MOD_RES 10: note = Phg
  MOD_RES 11: note = Nvl
  REGION 1..11: note = C-term NH2
YENGYWEYPGV

SEQ ID NO: 116 - protein, 10 aa, synthetic construct
  REGION 1..10: note = Description of Artificial Sequence: Synthetic peptide
  REGION 1..10: note = N-term heptanoyl
  REGION 1..9: note = misc_feature - Bridging moiety between residues
  MOD_RES 2: note = Phg
  MOD_RES 4: note = 7-azatryptophan
  MOD_RES 7: note = (N-Me)Ser
  MOD_RES 10: note = Nvl
  REGION 1..10: note = C-term NH2
CGTWEYSACV

SEQ ID NO: 117 - protein, 11 aa, synthetic construct
  REGION 1..11: note = Description of Artificial Sequence: Synthetic peptide
  REGION 1..11: note = N-term Ac
  MOD_RES 1: note = Nvl
  REGION 2..10: note = misc_feature - Bridging moiety between residues
  MOD_RES 3: note = Phg
  MOD_RES 5: note = 7-azatryptophan
  MOD_RES 11: note = Nvl
  REGION 1..11: note = C-term NH2
VCGTWEYSACV

SEQ ID NO: 118 - protein, 11 aa, synthetic construct
  REGION 1..11: note = Description of Artificial Sequence: Synthetic peptide
  REGION 1..11: note = N-term Ac
  MOD_RES 1: note = Nvl
  REGION 2..10: note = misc_feature - Bridging moiety between residues
  MOD_RES 3: note = Phg
  MOD_RES 5: note = (5-F)Trp
  MOD_RES 8: note = (N-Me)Ser
  MOD_RES 11: note = Nvl
  REGION 1..11: note = C-term NH2
VCGTWEYSACV

SEQ ID NO: 119 - protein, 11 aa, synthetic construct
  REGION 1..11: note = Description of Artificial Sequence: Synthetic peptide
  REGION 1..11: note = N-term Ac
  MOD_RES 1: note = Nvl
  REGION 2..10: note = misc_feature - Bridging moiety between residues
  MOD_RES 5: note = 7-azatryptophan
  MOD_RES 8: note = (N-Me)Ser
  MOD_RES 11: note = Nvl
  REGION 1..11: note = C-term NH2
VCFTWEYSACV

SEQ ID NO: 120 - protein, 11 aa, synthetic construct
  REGION 1..11: note = Description of Artificial Sequence: Synthetic peptide
  REGION 1..11: note = N-term Ac
  MOD_RES 1: note = Nvl
  REGION 2..10: note = misc_feature - Bridging moiety between residues
  MOD_RES 3: note = D-Chg
  MOD_RES 5: note = 7-azatryptophan
  MOD_RES 8: note = (N-Me)Ser
  MOD_RES 11: note = Nvl
  REGION 1..11: note = C-term NH2
VCGTWEYSACV

SEQ ID NO: 121 - protein, 11 aa, synthetic construct
  REGION 1..11: note = Description of Artificial Sequence: Synthetic peptide
  REGION 1..11: note = N-term Ac
  MOD_RES 4: note = Tbg
  MOD_RES 6: note = (5-MeO)Trp
  MOD_RES 10: note = Phg
  MOD_RES 11: note = Nvl
  REGION 1..11: note = C-term NH2
YENGYWEYPGV

SEQ ID NO: 122 - protein, 11 aa, synthetic construct
  REGION 1..11: note = Description of Artificial Sequence: Synthetic peptide
  REGION 1..11: note = N-term Ac
  MOD_RES 1: note = Nvl
  REGION 2..10: note = misc_feature - Bridging moiety between residues
  MOD_RES 3: note = Phg
  MOD_RES 5: note = 7-azatryptophan
  MOD_RES 8: note = (N-Me)Ser
  MOD_RES 11: note = Nvl
  REGION 1..11: note = C-term NH2
VCGTWDYSACV

SEQ ID NO: 123 - protein, 11 aa, synthetic construct
  REGION 1..11: note = Description of Artificial Sequence: Synthetic peptide
  REGION 1..11: note = N-term Ac
  MOD_RES 1: note = Nvl
  REGION 2..10: note = misc_feature - Bridging moiety between residues
  MOD_RES 3: note = Phg
  MOD_RES 5: note = 7-azatryptophan
  MOD_RES 8: note = (N-Me)Ser
  MOD_RES 11: note = Nvl
  REGION 1..11: note = C-term NH2
VCGTWQYSACV

SEQ ID NO: 124 - protein, 11 aa, synthetic construct
  REGION 1..11: note = Description of Artificial Sequence: Synthetic peptide
  REGION 1..11: note = N-term Ac
  MOD_RES 1: note = Nvl
  REGION 2..10: note = misc_feature - Bridging moiety between residues
  MOD_RES 3: note = Phg
  MOD_RES 5: note = 7-azatryptophan
  MOD_RES 8: note = (N-Me)Ser
  MOD_RES 11: note = Nvl
  REGION 1..11: note = C-term NH2
VCGTWNYSACV

SEQ ID NO: 125 - protein, 12 aa, synthetic construct
  REGION 1..12: note = Description of Artificial Sequence: Synthetic peptide
  REGION 1..12: note = N-term Ac
  MOD_RES 1: note = Nvl
  REGION 2..10: note = misc_feature - Bridging moiety between residues
  MOD_RES 3: note = Phg
  MOD_RES 5: note = 7-azatryptophan
  MOD_RES 8: note = (N-Me)Ser
  MOD_RES 12: note = Nvl
  REGION 1..12: note = C-term NH2
VCGTWEYSHGCV

SEQ ID NO: 126 - protein, 11 aa, synthetic construct
  REGION 1..11: note = Description of Artificial Sequence: Synthetic peptide
  REGION 1..11: note = N-term Ac
  MOD_RES 1: note = Nvl
  REGION 2..10: note = misc_feature - Bridging moiety between residues
  MOD_RES 3: note = Phg
  MOD_RES 5: note = 1-Me-Trp
  MOD_RES 8: note = (N-Me)Ser
  MOD_RES 11: note = Nvl
  REGION 1..11: note = C-term NH2
VCGTWEYSACV

SEQ ID NO: 127 - protein, 11 aa, synthetic construct
  REGION 1..11: note = Description of Artificial Sequence: Synthetic peptide
  REGION 1..11: note = N-term Ac
  MOD_RES 4: note = Tbg
  MOD_RES 6: note = D-Trp
  MOD_RES 10: note = Phg
  MOD_RES 11: note = Nvl
  REGION 1..11: note = C-term NH2
YENGYWEYPGV

SEQ ID NO: 128 - protein, 10 aa, synthetic construct
  REGION 1..10: note = Description of Artificial Sequence: Synthetic peptide
  REGION 1..10: note = N-term Ac
  MOD_RES 5: note = D-Trp
  MOD_RES 9: note = Phg
  MOD_RES 10: note = Nvl
  REGION 1..10: note = C-term NH2
YENYWEYPGV

SEQ ID NO: 129 - protein, 11 aa, synthetic construct
  REGION 1..11: note = Description of Artificial Sequence: Synthetic peptide
  REGION 1..11: note = N-term Ac
  MOD_RES 4: note = Tbg
  MOD_RES 6: note = 7-azatryptophan
  MOD_RES 7: note = D-Glu
  MOD_RES 10: note = Phg
  MOD_RES 11: note = Nvl
  REGION 1..11: note = C-term NH2
YENGYWEYPGV

SEQ ID NO: 130 - protein, 11 aa, synthetic construct
  REGION 1..11: note = Description of Artificial Sequence: Synthetic peptide
  REGION 1..11: note = N-term Ac
  REGION 1..6: note = misc_feature - Bridging moiety between residues
  REGION 1..11: note = C-term NH2
CVERFCVYWEF

SEQ ID NO: 131 - protein, 9 aa, synthetic construct
  REGION 1..9: note = Description of Artificial Sequence: Synthetic peptide
  REGION 1..9: note = N-term Ac
  REGION 1..6: note = misc_feature - Bridging moiety between residues
  REGION 1..9: note = C-term NH2
CVERFCWEF

SEQ ID NO: 132 - protein, 13 aa, synthetic construct
  REGION 1..13: note = Description of Artificial Sequence: Synthetic peptide
  REGION 1..13: note = N-term Ac
  MOD_RES 1: note = Nvl
  MOD_RES 6: note = Tbg
  MOD_RES 12: note = Phg
  MOD_RES 13: note = Tbg
  REGION 1..13: note = C-term NH2
VCYNNGECEYPGG

SEQ ID NO: 133 - protein, 13 aa, synthetic construct
  REGION 1..13: note = Description of Artificial Sequence: Synthetic peptide
  REGION 1..13: note = N-term Ac
  MOD_RES 1: note = Nvl
  REGION 2..8: note = misc_feature - Bridging moiety between residues
  MOD_RES 6: note = Tbg
  MOD_RES 12: note = Phg
  MOD_RES 13: note = Tbg
  REGION 1..13: note = C-term NH2
VCYNNGECEYPGG

SEQ ID NO: 134 - protein, 13 aa, synthetic construct
  REGION 1..13: note = Description of Artificial Sequence: Synthetic peptide
  REGION 1..13: note = N-term Ac
  MOD_RES 1..2: note = Nvl
  MOD_RES 6: note = Tbg
  MOD_RES 7: note = (N-Me)Tyr
  MOD_RES 8: note = 7-azatryptophan
  MOD_RES 12: note = Chg
  MOD_RES 13: note = Nvl
  REGION 1..13: note = C-term NH2
VVYENGYWEYPGV

SEQ ID NO: 135 - protein, 11 aa, synthetic construct
  REGION 1..11: note = Description of Artificial Sequence: Synthetic peptide
  REGION 1..11: note = N-term Ac
  MOD_RES 1: note = Nvl
  REGION 2..10: note = misc_feature - Bridging moiety between residues
  MOD_RES 3: note = Phg
  MOD_RES 6: note = Asp(T)
  MOD_RES 8: note = (N-Me)Ser
  MOD_RES 11: note = Nvl
  REGION 1..11: note = C-term NH2
VCGTWXYSHCV

SEQ ID NO: 136 - protein, 11 aa, synthetic construct
  REGION 1..11: note = Description of Artificial Sequence: Synthetic peptide
  REGION 1..11: note = N-term Ac
  MOD_RES 1: note = Nvl
  REGION 2..10: note = misc_feature - Bridging moiety between residues
  MOD_RES 3: note = Phg
  MOD_RES 5: note = D-Trp
  MOD_RES 8: note = (N-Me)Ser
  MOD_RES 11: note = Nvl
  REGION 1..11: note = C-term NH2
VCGTWEYSHCV

SEQ ID NO: 137 - protein, 11 aa, synthetic construct
  REGION 1..11: note = Description of Artificial Sequence: Synthetic peptide
  REGION 1..11: note = N-term heptanoyl
  MOD_RES 1: note = Nvl
  REGION 2..10: note = misc_feature - Bridging moiety between residues
  MOD_RES 3: note = D-Phg
  MOD_RES 5: note = azaTrp
  MOD_RES 8: note = (N-Me)Ser
  MOD_RES 11: note = Nvl
  REGION 1..11: note = C-term NH2
VCGTWEYSACV

SEQ ID NO: 138 - protein, 10 aa, synthetic construct
  REGION 1..10: note = Description of Artificial Sequence: Synthetic peptide
  REGION 1..10: note = N-term heptanoyl
  REGION 1..9: note = misc_feature - Bridging moiety between residues
  MOD_RES 2: note = D-Phg
  MOD_RES 4: note = azaTrp
  MOD_RES 7: note = (N-Me)Ser
  MOD_RES 10: note = Nvl
  REGION 1..10: note = C-term NH2
CGTWEYSACV

SEQ ID NO: 139 - protein, 12 aa, synthetic construct
  REGION 1..12: note = Description of Artificial Sequence: Synthetic peptide
  REGION 1..12: note = N-term Ac
  REGION 1..6: note = misc_feature - Bridging moiety between residues
  MOD_RES 8: note = Tbg
  REGION 1..12: note = C-term NH2
CVERFCDGYWEF

SEQ ID NO: 140 - protein, 12 aa, synthetic construct
  REGION 1..12: note = Description of Artificial Sequence: Synthetic peptide
  REGION 1..12: note = N-term Ac
  REGION 1..6: note = misc_feature - Bridging moiety between residues
  MOD_RES 2: note = Tbg
  MOD_RES 8: note = Tbg
  REGION 1..12: note = C-term NH2
CGERFCDGYWEF

SEQ ID NO: 141 - protein, 13 aa, synthetic construct
  REGION 1..13: note = Description of Artificial Sequence: Synthetic peptide
  REGION 1..13: note = N-term Ac
  REGION 1..6: note = misc_feature - Bridging moiety between residues
  REGION 1..13: note = C-term NH2
CVERFCDVYWEYP

SEQ ID NO: 142 - protein, 13 aa, synthetic construct
  REGION 1..13: note = Description of Artificial Sequence: Synthetic peptide
  REGION 1..13: note = N-term Ac
  REGION 1..6: note = misc_feature - Bridging moiety between residues
  REGION 1..13: note = C-term NH2
CVERFCDVYWEFP

SEQ ID NO: 143 - protein, 13 aa, synthetic construct
  REGION 1..13: note = Description of Artificial Sequence: Synthetic peptide
  REGION 1..13: note = N-term Ac
  REGION 1..6: note = misc_feature - Bridging moiety between residues
  MOD_RES 10: note = azaTrp
  REGION 1..13: note = C-term NH2
CVERFCDVYWEYP

SEQ ID NO: 144 - protein, 13 aa, synthetic construct
  REGION 1..13: note = Description of Artificial Sequence: Synthetic peptide
  REGION 1..13: note = N-term Ac
  REGION 1..6: note = misc_feature - Bridging moiety between residues
  MOD_RES 8: note = Tbg
  REGION 1..13: note = C-term NH2
CVERFCDGYWEYP

SEQ ID NO: 145 - protein, 15 aa, synthetic construct
  REGION 1..15: note = Description of Artificial Sequence: Synthetic peptide
  REGION 1..15: note = N-term Ac
  REGION 1..6: note = misc_feature - Bridging moiety between residues
  MOD_RES 8: note = Tbg
  MOD_RES 10: note = azaTrp
  MOD_RES 14: note = Phg
  MOD_RES 15: note = Nvl
  REGION 1..15: note = C-term NH2
CVERFCDGYWEYPGV

SEQ ID NO: 146 - protein, 15 aa, synthetic construct
  REGION 1..15: note = Description of Artificial Sequence: Synthetic peptide
  REGION 1..15: note = N-term Ac
  REGION 1..6: note = misc_feature - Bridging moiety between residues
  MOD_RES 8: note = Tbg
  MOD_RES 10: note = azaTrp
  MOD_RES 14: note = D-Phg
  MOD_RES 15: note = Nvl
  REGION 1..15: note = C-term NH2
CVERFCDGYWEYPGV

SEQ ID NO: 147 - protein, 12 aa, synthetic construct
  REGION 1..12: note = Description of Artificial Sequence: Synthetic peptide
  REGION 1..12: note = N-term Ac
  REGION 1..6: note = misc_feature - Bridging moiety between residues
  MOD_RES 2: note = Tbg
  REGION 1..12: note = C-term NH2
CGERFCDVYWEF

SEQ ID NO: 148 - protein, 13 aa, synthetic construct
  REGION 1..13: note = Description of Artificial Sequence: Synthetic peptide
  REGION 1..13: note = N-term Ac
  REGION 1..6: note = misc_feature - Bridging moiety between residues
  MOD_RES 13: note = Propargyl-Gly
  REGION 1..13: note = C-term NH2
CVERFCDVYWEFG

SEQ ID NO: 149 - protein, 15 aa, synthetic construct
  REGION 1..15: note = Description of Artificial Sequence: Synthetic peptide
  REGION 1..15: note = N-term Ac
  REGION 1..6: note = misc_feature - Bridging moiety between residues
  MOD_RES 8: note = Tbg
  MOD_RES 14: note = Phg
  MOD_RES 15: note = Nvl
  REGION 1..15: note = C-term NH2
CAERFCDGYWEYPGV

SEQ ID NO: 150 - protein, 15 aa, synthetic construct
  REGION 1..15: note = Description of Artificial Sequence: Synthetic peptide
  REGION 1..15: note = N-term Ac
  REGION 1..6: note = misc_feature - Bridging moiety between residues
  MOD_RES 8: note = Tbg
  MOD_RES 14: note = D-Phg
  MOD_RES 15: note = Nvl
  REGION 1..15: note = C-term NH2
CAERFCDGYWEYPGV

SEQ ID NO: 151 - protein, 15 aa, synthetic construct
  REGION 1..15: note = Description of Artificial Sequence: Synthetic peptide
  REGION 1..15: note = N-term Ac
  REGION 1..6: note = misc_feature - Bridging moiety between residues
  MOD_RES 8: note = Tbg
  MOD_RES 10: note = azaTrp
  MOD_RES 14: note = Phg
  MOD_RES 15: note = Nvl
  REGION 1..15: note = C-term NH2
CVARFCDGYWEYPGV

SEQ ID NO: 152 - protein, 15 aa, synthetic construct
  REGION 1..15: note = Description of Artificial Sequence: Synthetic peptide
  REGION 1..15: note = N-term Ac
  REGION 1..6: note = misc_feature - Bridging moiety between residues
  MOD_RES 8: note = Tbg
  MOD_RES 10: note = azaTrp
  MOD_RES 14: note = D-Phg
  MOD_RES 15: note = Nvl
  REGION 1..15: note = C-term NH2
CVARFCDGYWEYPGV

SEQ ID NO: 153 - protein, 15 aa, synthetic construct
  REGION 1..15: note = Description of Artificial Sequence: Synthetic peptide
  REGION 1..15: note = N-term Ac
  REGION 1..6: note = misc_feature - Bridging moiety between residues
  MOD_RES 8: note = Tbg
  MOD_RES 10: note = azaTrp
  MOD_RES 14: note = Chg
  MOD_RES 15: note = Nvl
  REGION 1..15: note = C-term NH2
CVERFCDGYWEYPGV

SEQ ID NO: 154 - protein, 15 aa, synthetic construct
  REGION 1..15: note = Description of Artificial Sequence: Synthetic peptide
  REGION 1..15: note = N-term Ac
  REGION 1..6: note = misc_feature - Bridging moiety between residues
  MOD_RES 8: note = Tbg
  MOD_RES 10: note = azaTrp
  MOD_RES 14: note = Phg
  MOD_RES 15: note = Nvl
  REGION 1..15: note = C-term NH2
CVEAFCDGYWEYPGV

SEQ ID NO: 155 - protein, 15 aa, synthetic construct
  REGION 1..15: note = Description of Artificial Sequence: Synthetic peptide
  REGION 1..15: note = N-term Ac
  REGION 1..6: note = misc_feature - Bridging moiety between residues
  MOD_RES 8: note = Tbg
  MOD_RES 10: note = azaTrp
  MOD_RES 14: note = D-Phg
  MOD_RES 15: note = Nvl
  REGION 1..15: note = C-term NH2
CVEAFCDGYWEYPGV

SEQ ID NO: 156 - protein, 15 aa, synthetic construct
  REGION 1..15: note = Description of Artificial Sequence: Synthetic peptide
  REGION 1..15: note = N-term Ac
  REGION 1..6: note = misc_feature - Bridging moiety between residues
  MOD_RES 8: note = Tbg
  MOD_RES 10: note = azaTrp
  MOD_RES 14: note = Phg
  MOD_RES 15: note = Nvl
  REGION 1..15: note = C-term NH2
CVERACDGYWEYPGV

SEQ ID NO: 157 - protein, 15 aa, synthetic construct
  REGION 1..15: note = Description of Artificial Sequence: Synthetic peptide
  REGION 1..15: note = N-term Ac
  REGION 1..6: note = misc_feature - Bridging moiety between residues
  MOD_RES 8: note = Tbg
  MOD_RES 10: note = azaTrp
  MOD_RES 14: note = D-Phg
  MOD_RES 15: note = Nvl
  REGION 1..15: note = C-term NH2
CVERACDGYWEYPGV

SEQ ID NO: 158 - protein, 15 aa, synthetic construct
  REGION 1..15: note = Description of Artificial Sequence: Synthetic peptide
  REGION 1..15: note = N-term Ac
  REGION 1..6: note = misc_feature - Bridging moiety between residues
  MOD_RES 8: note = Tbg
  MOD_RES 10: note = azaTrp
  MOD_RES 14: note = Phg
  MOD_RES 15: note = Nvl
  REGION 1..15: note = C-term NH2
CVERFCAGYWEYPGV

SEQ ID NO: 159 - protein, 15 aa, synthetic construct
  REGION 1..15: note = Description of Artificial Sequence: Synthetic peptide
  REGION 1..15: note = N-term Ac
  REGION 1..6: note = misc_feature - Bridging moiety between residues
  MOD_RES 8: note = Tbg
  MOD_RES 10: note = azaTrp
  MOD_RES 14: note = D-Phg
  MOD_RES 15: note = Nvl
  REGION 1..15: note = C-term NH2
CVERFCAGYWEYPGV

SEQ ID NO: 160 - protein, 15 aa, synthetic construct
  REGION 1..15: note = Description of Artificial Sequence: Synthetic peptide
  REGION 1..6: note = misc_feature - Bridging moiety between residues
  MOD_RES 1: note = (des-amino)Cys
  MOD_RES 8: note = Tbg
  MOD_RES 10: note = azaTrp
  MOD_RES 14: note = Phg
  MOD_RES 15: note = Nvl
  REGION 1..15: note = C-term NH2
CVERFCDGYWEYPGV

SEQ ID NO: 161 - protein, 15 aa, synthetic construct
  REGION 1..15: note = Description of Artificial Sequence: Synthetic peptide
  REGION 1..6: note = misc_feature - Bridging moiety between residues
  MOD_RES 1: note = (des-amino)Cys
  MOD_RES 8: note = Tbg
  MOD_RES 10: note = azaTrp
  MOD_RES 14: note = D-Phg
  MOD_RES 15: note = Nvl
  REGION 1..15: note = C-term NH2
CVERFCDGYWEYPGV

SEQ ID NO: 162 - protein, 15 aa, synthetic construct
  REGION 1..15: note = Description of Artificial Sequence: Synthetic peptide
  REGION 1..15: note = N-term Ac
  REGION 1..6: note = misc_feature - Bridging moiety between residues
  MOD_RES 8: note = Tbg
  MOD_RES 10: note = azaTrp
  MOD_RES 14: note = Phg
  REGION 1..15: note = C-term NH2
CAERFCDGYWEYPGK

SEQ ID NO: 163 - protein, 15 aa, synthetic construct
  REGION 1..15: note = Description of Artificial Sequence: Synthetic peptide
  REGION 1..15: note = N-term Ac
  REGION 1..6: note = misc_feature - Bridging moiety between residues
  MOD_RES 8: note = Tbg
  MOD_RES 10: note = azaTrp
  MOD_RES 14: note = D-Phg
  REGION 1..15: note = C-term NH2
CAERFCDGYWEYPGK

SEQ ID NO: 164 - protein, 15 aa, synthetic construct
  REGION 1..15: note = Description of Artificial Sequence: Synthetic peptide
  REGION 1..15: note = N-term Ac
  REGION 1..6: note = misc_feature - Cyclic
  MOD_RES 8: note = Tbg
  MOD_RES 10: note = azaTrp
  MOD_RES 14: note = Phg
  MOD_RES 15: note = Nvl
  REGION 1..15: note = C-term NH2
CVERFCDGYWEYPGV

SEQ ID NO: 165 - protein, 15 aa, synthetic construct
  REGION 1..15: note = Description of Artificial Sequence: Synthetic peptide
  REGION 1..15: note = N-term Ac
  REGION 1..6: note = misc_feature - Bridging moiety between residues
  MOD_RES 8: note = Tbg
  MOD_RES 10: note = azaTrp
  MOD_RES 14: note = Phg
  MOD_RES 15: note = Lys-C12
  REGION 1..15: note = C-term NH2
CAERFCDGYWEYPGK

SEQ ID NO: 166 - protein, 15 aa, synthetic construct
  REGION 1..15: note = Description of Artificial Sequence: Synthetic peptide
  REGION 1..15: note = N-term Ac
  REGION 1..6: note = misc_feature - Bridging moiety between residues
  MOD_RES 8: note = Tbg
  MOD_RES 10: note = azaTrp
  MOD_RES 14: note = Phg
  MOD_RES 15: note = Lys-C10
  REGION 1..15: note = C-term NH2
CAERFCDGYWEYPGK

SEQ ID NO: 167 - protein, 15 aa, synthetic construct
  REGION 1..15: note = Description of Artificial Sequence: Synthetic peptide
  REGION 1..15: note = N-term Ac
  REGION 1..6: note = misc_feature - Bridging moiety between residues
  MOD_RES 8: note = Tbg
  MOD_RES 10: note = azaTrp
  MOD_RES 14: note = Phg
  MOD_RES 15: note = Lys-C8
  REGION 1..15: note = C-term NH2
CAERFCDGYWEYPGK

SEQ ID NO: 168 - protein, 15 aa, synthetic construct
  REGION 1..15: note = Description of Artificial Sequence: Synthetic peptide
  REGION 1..15: note = N-term Ac
  REGION 1..6: note = misc_feature - Bridging moiety between residues
  MOD_RES 7: note = (alpha-methyl)Asp
  MOD_RES 8: note = Tbg
  MOD_RES 10: note = azaTrp
  MOD_RES 14: note = Chg
  MOD_RES 15: note = Nvl
  REGION 1..15: note = C-term NH2
CVERFCDGYWEYPGV

SEQ ID NO: 169 - protein, 15 aa, synthetic construct
  REGION 1..15: note = Description of Artificial Sequence: Synthetic peptide
  REGION 1..15: note = N-term Ac
  REGION 1..6: note = misc_feature - Bridging moiety between residues
  MOD_RES 7: note = Asp(T)
  MOD_RES 8: note = Tbg
  MOD_RES 10: note = azaTrp
  MOD_RES 14: note = Chg
  MOD_RES 15: note = Nvl
  REGION 1..15: note = C-term NH2
CVERFCXGYWEYPGV

SEQ ID NO: 170 - protein, 15 aa, synthetic construct
  REGION 1..15: note = Description of Artificial Sequence: Synthetic peptide
  REGION 1..15: note = N-term Ac
  REGION 1..6: note = misc_feature - Cyclic
  MOD_RES 8: note = Tbg
  MOD_RES 10: note = azaTrp
  MOD_RES 14: note = Chg
  MOD_RES 15: note = Nvl
  REGION 1..15: note = C-term NH2
KVERFDDGYWEYPGV

SEQ ID NO: 171 - protein, 15 aa, synthetic construct
  REGION 1..15: note = Description of Artificial Sequence: Synthetic peptide
  REGION 1..15: note = N-term Ac
  REGION 1..6: note = misc_feature - Bridging moiety between residues
  MOD_RES 8: note = Tbg
  MOD_RES 10: note = azaTrp
  MOD_RES 14: note = Phg
CAERFCDGYWEYPGK

SEQ ID NO: 172 - protein, 15 aa, synthetic construct
  REGION 1..15: note = Description of Artificial Sequence: Synthetic peptide
  REGION 1..15: note = N-term Ac
  REGION 1..6: note = misc_feature - Bridging moiety between residues
  MOD_RES 8: note = Tbg
  MOD_RES 10: note = azaTrp
  MOD_RES 14: note = Phg
  MOD_RES 15: note = Lys-C12
CAERFCDGYWEYPGK

SEQ ID NO: 173 - protein, 15 aa, synthetic construct
  REGION 1..15: note = Description of Artificial Sequence: Synthetic peptide
  REGION 1..15: note = N-term Ac
  REGION 1..6: note = misc_feature - Bridging moiety between residues
  MOD_RES 7: note = (N-Me)Asp
  MOD_RES 8: note = Tbg
  MOD_RES 10: note = azaTrp
  MOD_RES 14: note = Chg
  MOD_RES 15: note = Nvl
  REGION 1..15: note = C-term NH2
CVERFCDGYWEYPGV

SEQ ID NO: 174 - protein, 15 aa, synthetic construct
  REGION 1..15: note = Description of Artificial Sequence: Synthetic peptide
  REGION 1..15: note = N-term Ac
  REGION 1..6: note = misc_feature - Cyclic
  MOD_RES 8: note = Tbg
  MOD_RES 10: note = azaTrp
  MOD_RES 14: note = Chg
  MOD_RES 15: note = Nvl
KVERFDDGYWEYPGV

SEQ ID NO: 175 - protein, 15 aa, synthetic construct
  REGION 1..15: note = Description of Artificial Sequence: Synthetic peptide
  REGION 1..15: note = N-term Ac
  REGION 1..6: note = misc_feature - Cyclic
  MOD_RES 7: note = Asp(T)
  MOD_RES 8: note = Tbg
  MOD_RES 10: note = azaTrp
  MOD_RES 14: note = Chg
  MOD_RES 15: note = Nvl
KVERFDXGYWEYPGV

SEQ ID NO: 176 - protein, 15 aa, synthetic construct
  REGION 1..15: note = Description of Artificial Sequence: Synthetic peptide
  REGION 1..15: note = N-term Ac
  REGION 1..6: note = misc_feature - Cyclic
  MOD_RES 8: note = Tbg
  MOD_RES 10: note = azaTrp
  MOD_RES 14: note = Chg
  MOD_RES 15: note = N-epsilon-(PEG2-gamma-glutamic acid-N-alpha-octadecanedioic acid) lysine
KVERFDDGYWEYPGK

SEQ ID NO: 177 - protein, 15 aa, synthetic construct
  REGION 1..15: note = Description of Artificial Sequence: Synthetic peptide
  REGION 1..15: note = N-term Ac
  REGION 1..6: note = misc_feature - Cyclic
  MOD_RES 7: note = (N-Me)Asp
  MOD_RES 8: note = Tbg
  MOD_RES 10: note = azaTrp
  MOD_RES 14: note = Chg
  MOD_RES 15: note = Nvl
KVERFDDGYWEYPGV

SEQ ID NO: 178 - protein, 15 aa, synthetic construct
  REGION 1..15: note = Description of Artificial Sequence: Synthetic peptide
  REGION 1..15: note = N-term Ac
  REGION 1..6: note = misc_feature - Bridging moiety between residues
  MOD_RES 8: note = Tbg
  MOD_RES 10: note = azaTrp
  MOD_RES 14: note = Chg
  MOD_RES 15: note = Nvl
CVERFCDGYWEWPGV

SEQ ID NO: 179 - protein, 15 aa, synthetic construct
  REGION 1..15: note = Description of Artificial Sequence: Synthetic peptide
  REGION 1..15: note = N-term Ac
  REGION 1..6: note = misc_feature - Bridging moiety between residues
  MOD_RES 8: note = Tbg
  MOD_RES 10: note = azaTrp
  MOD_RES 12: note = (homo)Phe
  MOD_RES 14: note = Chg
  MOD_RES 15: note = Nvl
CVERFCDGYWEFPGV

SEQ ID NO: 180 - protein, 15 aa, synthetic construct
  REGION 1..15: note = Description of Artificial Sequence: Synthetic peptide
  REGION 1..15: note = N-term Ac
  REGION 1..6: note = misc_feature - Bridging moiety between residues
  MOD_RES 8: note = Tbg
  MOD_RES 10: note = azaTrp
  MOD_RES 12: note = (m-Cl-homo)Phe
  MOD_RES 14: note = Chg
  MOD_RES 15: note = Nvl
CVERFCDGYWEFPGV

SEQ ID NO: 181 - protein, 15 aa, synthetic construct
  REGION 1..15: note = Description of Artificial Sequence: Synthetic peptide
  REGION 1..15: note = N-term Ac
  REGION 1..6: note = misc_feature - Bridging moiety between residues
  MOD_RES 8: note = Tbg
  MOD_RES 10: note = azaTrp
  MOD_RES 12: note = 2Nal
  MOD_RES 14: note = Chg
  MOD_RES 15: note = Nvl
CVERFCDGYWEAPGV

SEQ ID NO: 182 - protein, 15 aa, synthetic construct
  REGION 1..15: note = Description of Artificial Sequence: Synthetic peptide
  REGION 1..15: note = N-term Ac
  REGION 1..6: note = misc_feature - Bridging moiety between residues
  MOD_RES 8: note = Tbg
  MOD_RES 10: note = (3-aminomethyl)Phe
  MOD_RES 14: note = Chg
  MOD_RES 15: note = Nvl
CVERFCDGYFEYPGV

SEQ ID NO: 183 - protein, 15 aa, synthetic construct
  REGION 1..15: note = Description of Artificial Sequence: Synthetic peptide
  REGION 1..15: note = N-term Ac
  REGION 1..6: note = misc_feature - Cyclo-triazolyl linkage between residues
  MOD_RES 1: note = (S)-2-amino-5-azidopentanoic acid
  MOD_RES 6: note = (S)-2-aminopent-4-ynoic acid
  MOD_RES 8: note = Tbg
  MOD_RES 10: note = azaTrp
  MOD_RES 14: note = Chg
  MOD_RES 15: note = Nvl
XVERFXDGYWEYPGV

SEQ ID NO: 184 - protein, 15 aa, synthetic construct
  REGION 1..15: note = Description of Artificial Sequence: Synthetic peptide
  REGION 1..15: note = N-term Ac
  REGION 1..6: note = misc_feature - Cyclic
  MOD_RES 7: note = (N-Me)Asp
  MOD_RES 8: note = Tbg
  MOD_RES 10: note = azaTrp
  MOD_RES 14: note = Chg
  MOD_RES 15: note = Lys-C16
KVERFDDGYWEYPGK

SEQ ID NO: 185 - protein, 14 aa, synthetic construct
  REGION 1..14: note = Description of Artificial Sequence: Synthetic peptide
  REGION 1..5: note = misc_feature - Cyclo-thioalkyl linkage between residues
  MOD_RES 1: note = Chloroacetic acid-Val
  MOD_RES 7: note = Tbg
  MOD_RES 9: note = azaTrp
  MOD_RES 13: note = Chg
  MOD_RES 14: note = Nvl
VERFCDGYWEYPGV

SEQ ID NO: 186 - protein, 15 aa, synthetic construct
  REGION 1..15: note = Description of Artificial Sequence: Synthetic peptide
  REGION 1..15: note = N-term Ac
  REGION 1..6: note = misc_feature - Bridging moiety between residues
  MOD_RES 7: note = Cle
  MOD_RES 8: note = Tbg
  MOD_RES 10: note = azaTrp
  MOD_RES 14: note = Chg
  MOD_RES 15: note = Nvl
CVERFCLGYWEYPGV

SEQ ID NO: 187 - protein, 15 aa, synthetic construct
  REGION 1..15: note = Description of Artificial Sequence: Synthetic peptide
  REGION 1..15: note = N-term Ac
  REGION 1..6: note = misc_feature - Bridging moiety between residues
  MOD_RES 7: note = Ac-Pyran
  MOD_RES 8: note = Tbg
  MOD_RES 10: note = azaTrp
  MOD_RES 14: note = Chg
  MOD_RES 15: note = Nvl
CVERFCXGYWEYPGV

SEQ ID NO: 188 - protein, 15 aa, synthetic construct
  REGION 1..15: note = Description of Artificial Sequence: Synthetic peptide
  REGION 1..15: note = N-term Ac
  REGION 1..6: note = misc_feature - Bridging moiety between residues
  MOD_RES 8: note = Tbg
  MOD_RES 10: note = azaTrp
  MOD_RES 12: note = (3-aminomethyl)Phe
  MOD_RES 14: note = Chg
  MOD_RES 15: note = Nvl
CVERFCDGYWEFPGV

SEQ ID NO: 189 - protein, 15 aa, synthetic construct
  REGION 1..15: note = Description of Artificial Sequence: Synthetic peptide
  REGION 1..15: note = N-term Ac
  REGION 1..6: note = misc_feature - Cyclo-olefinyl linkage between residues
  MOD_RES 1: note = (S)-2-aminohept-6-enoic acid
  MOD_RES 6: note = (S)-2-aminopent-4-enoic acid
  MOD_RES 8: note = Tbg
  MOD_RES 10: note = azaTrp
  MOD_RES 14: note = Chg
  MOD_RES 15: note = Nvl
XVERFXDGYWEYPGV

SEQ ID NO: 190 - protein, 15 aa, synthetic construct
  REGION 1..15: note = Description of Artificial Sequence: Synthetic peptide
  REGION 1..15: note = N-term Ac
  REGION 1..6: note = misc_feature - Bridging moiety between residues
  MOD_RES 8: note = Tbg
  MOD_RES 10: note = azaTrp
  MOD_RES 14: note = Phg
  MOD_RES 15: note = Lys-C16
CAERFCDGYWEYPGK

SEQ ID NO: 191 - protein, 15 aa, synthetic construct
  REGION 1..15: note = Description of Artificial Sequence: Synthetic peptide
  REGION 1..15: note = N-term Ac
  REGION 1..6: note = misc_feature - Cyclic
  MOD_RES 7: note = (N-Me)Asp
  MOD_RES 8: note = Tbg
  MOD_RES 10: note = azaTrp
  MOD_RES 14: note = Chg
  MOD_RES 15: note = N-epsilon-(PEG2-gamma-glutamic acid-N-alpha-octadecanedioic acid) lysine
KVERFDDGYWEYPGK

SEQ ID NO: 192 - protein, 15 aa, synthetic construct
  REGION 1..15: note = Description of Artificial Sequence: Synthetic peptide
  REGION 1..15: note = N-term Ac
  REGION 1..6: note = misc_feature - Cyclic
  MOD_RES 7: note = (N-Me)Asp
  MOD_RES 8: note = Tbg
  MOD_RES 10: note = azaTrp
  MOD_RES 14: note = Chg
KVERFDDGYWEYPGK

SEQ ID NO: 193 - protein, 15 aa, synthetic construct
  REGION 1..15: note = Description of Artificial Sequence: Synthetic peptide
  REGION 1..15: note = N-term Ac
  REGION 1..6: note = misc_feature - Cyclic
  MOD_RES 7: note = (N-Me)Asp
  MOD_RES 8: note = Tbg
  MOD_RES 10: note = azaTrp
  MOD_RES 14: note = Chg
  REGION 1..15: note = C-term NH2
KVERFDDGYWEYPGK

SEQ ID NO: 194 - protein, 15 aa, synthetic construct
  REGION 1..15: note = Description of Artificial Sequence: Synthetic peptide
  REGION 1..15: note = N-term Ac
  REGION 1..6: note = misc_feature - Cyclic
  MOD_RES 7: note = (N-Me)Asp
  MOD_RES 8: note = Tbg
  MOD_RES 10: note = azaTrp
  MOD_RES 14: note = Chg
  MOD_RES 15: note = N-epsilon-(PEG24-gamma-glutamic acid-N-alpha-hexadecanoyl)lysine
KVERFDDGYWEYPGK

SEQ ID NO: 195 - protein, 15 aa, synthetic construct
  REGION 1..15: note = Description of Artificial Sequence: Synthetic peptide
  REGION 1..15: note = N-term Ac
  REGION 1..6: note = misc_feature - Cyclic
  MOD_RES 7: note = (N-Me)Asp
  MOD_RES 8: note = Tbg
  MOD_RES 10: note = azaTrp
  MOD_RES 14: note = Chg
  MOD_RES 15: note = Lys-C16
  REGION 1..15: note = C-term NH2
KVERFDDGYWEYPGK

SEQ ID NO: 196 - protein, 15 aa, synthetic construct
  REGION 1..15: note = Description of Artificial Sequence: Synthetic peptide
  REGION 1..15: note = N-term Ac
  REGION 1..6: note = misc_feature - Cyclic
  MOD_RES 7: note = (N-Me)Asp
  MOD_RES 8: note = Tbg
  MOD_RES 14: note = Chg
  MOD_RES 15: note = Lys-C16
KVERFDDGYWEYPGK

SEQ ID NO: 197 - protein, 15 aa, synthetic construct
  REGION 1..15: note = Description of Artificial Sequence: Synthetic peptide
  REGION 1..15: note = N-term Ac
  REGION 1..6: note = misc_feature - Cyclic
  MOD_RES 7: note = (N-Me)Asp
  MOD_RES 8: note = Tbg
  MOD_RES 14: note = Chg
KVERFDDGYWEYPGK

SEQ ID NO: 198 - protein, 15 aa, synthetic construct
  REGION 1..15: note = Description of Artificial Sequence: Synthetic peptide
  REGION 1..15: note = N-term Ac
  REGION 1..6: note = misc_feature - Cyclic
  MOD_RES 7: note = (N-Me)Asp
  MOD_RES 8: note = Tbg
  MOD_RES 14: note = Chg
  MOD_RES 15: note = N-epsilon-1-(4,4-dimethyl-2,6-dioxocyclohex-1-ylidene)- 3-methylbutyl-L-lysine
KVERFDDGYWEYPGK

SEQ ID NO: 199 - protein, 15 aa, synthetic construct
  REGION 1..15: note = Description of Artificial Sequence: Synthetic peptide
  REGION 1..6: note = misc_feature - Cyclic
  MOD_RES 1: note = (desamino)Cys
  MOD_RES 7: note = (N-Me)Asp
  MOD_RES 8: note = Tbg
  MOD_RES 10: note = azaTrp
  MOD_RES 14: note = Chg
  MOD_RES 15: note = Lys-C16
CVERFCDGYWEYPGK

SEQ ID NO: 200 - protein, 15 aa, synthetic construct
  REGION 1..15: note = Description of Artificial Sequence: Synthetic peptide
  REGION 1..6: note = misc_feature - Cyclic
  MOD_RES 1: note = (desamino)Cys
  MOD_RES 2: note = D-Ala
  MOD_RES 7: note = (N-Me)Asp
  MOD_RES 8: note = Tbg
  MOD_RES 10: note = azaTrp
  MOD_RES 14: note = Chg
  MOD_RES 15: note = Lys-C16
CAERFCDGYWEYPGK

SEQ ID NO: 201 - protein, 15 aa, synthetic construct
  REGION 1..15: note = Description of Artificial Sequence: Synthetic peptide
  REGION 1..15: note = N-term Ac
  REGION 1..6: note = misc_feature - Cyclic
  MOD_RES 7: note = (N-Me)Asp
  MOD_RES 8: note = Tbg
  MOD_RES 10: note = azaTrp
  MOD_RES 14: note = Aib
  MOD_RES 15: note = Lys-C16
KVERFDDGYWEYPXK

SEQ ID NO: 202 - protein, 19 aa, synthetic construct
  REGION 1..19: note = Description of Artificial Sequence: Synthetic peptide
  REGION 1..19: note = N-term Ac
  REGION 1..19: note = C-term NH2
RLIEDICLIPRWGCLWEDD

SEQ ID NO: 203 - protein, 20 aa, synthetic construct
  REGION 1..20: note = Description of Artificial Sequence: Synthetic peptide
  REGION 1..20: note = C-term NH2
QRLMEDICLPRWGCLWEDDF

SEQ ID NO: 204 - protein, 20 aa, synthetic construct
  REGION 1..20: note = Description of Artificial Sequence: Synthetic peptide
  REGION 1..20: note = N-term Ac
  REGION 1..20: note = C-term NH2
QRLIEDICLPRWGCLWEDDF

SEQ ID NO: 205 - protein, 16 aa, synthetic construct
  REGION 1..16: note = Description of Artificial Sequence: Synthetic peptide
RKKRRRESRKKRRRES

SEQ ID NO: 206 - protein, 9 aa, synthetic construct
  REGION 1..9: note = Description of Artificial Sequence: Synthetic peptide
RKKRRQRRR

SEQ ID NO: 207 - protein, 16 aa, synthetic construct
  REGION 1..16: note = Description of Artificial Sequence: Synthetic peptide
RQIKIWFQNRRMKWKK

SEQ ID NO: 208 - protein, 12 aa, synthetic construct
  REGION 1..12: note = Description of Artificial Sequence: Synthetic peptide
AAVLLPVLLAAP

SEQ ID NO: 209 - protein, 5 aa, synthetic construct
  REGION 1..5: note = Description of Artificial Sequence: Synthetic peptide
VPTLK

SEQ ID NO: 210 - protein, 12 aa, synthetic construct
  REGION 1..12: note = Description of Artificial Sequence: Synthetic peptide
PLILLRLLRGQF

SEQ ID NO: 211 - protein, 15 aa, synthetic construct
  REGION 1..15: note = Description of Artificial Sequence: Synthetic peptide
  REGION 1..15: note = N-term Ac
  REGION 1..6: note = misc_feature - Bridging moiety between residues
  MOD_RES 8: note = Tbg
  MOD_RES 10: note = azaTrp
  MOD_RES 14: note = Chg
  MOD_RES 15: note = Nvl
CVERFCDGYWEYPGV

SEQ ID NO: 212 - skipped